European Patent Specification EP 3 061 819 B1, published May 24, 2023. Title: Method for determining hemoglobin A1c and kit thereof. Applicant: Kikkoman Corporation. The sequence listing filed with the application follows.

SEQUENCE LISTING (204 sequences)

SEQ ID NO: 1 - protein, 437 aa, Coniochaeta sp. [sequence omitted]

SEQ ID NO: 2 - DNA, 1314 bp, Coniochaeta sp.
atgacgtcgaatcgtgcagatacaagggtgattgtcgtcggtggcggaggaacgattggttcctcgacagcgctgcatcttgtgaggagtggttatgctcccgcaaatatcacggtcttggacacatttgagattccatcggctcaatcagccggccatgatctcaacaagatcatgggaatacgactgcgcaacaaggtggacctgcaaatgagtctagaggctagacagatgtggaaggaggatgagttattccagcccttctttcacaataccggcagaatggactgcgaacacacgcctgagggtatcgaggacctgaaaaagcagtaccaggcactgcacgatgccggtgcgggtctggagaagactcatgcctggttggacaacgaggatgagatcttatccaagatgccgttgcttcaacgtgaccaaatacaaggatggaaagcaatatggagtcaagatggcggctggttagctgcggcaaaggccatcaatgcgatcggacagttcttgaaagaacgtggtgtaaagttcggattcggcggcgctggatccttcaagcaaccccttttcgacgatgaaggcacaacttgcattggcgttgagacggcagatggtaccaaatattacgctgacaaggtggtcttagcagctggcgcatggagcccaaccctggtggacctggaagatcaatgttgctcgaaggcttgggtgtatgctcatattcagttgacgcctgaagaggccgctgagtataagggtgtcccagttgtgtataatggcgaatttggcttcttctttgagcctgatgagtttggtgtaataaaggtgtgcgacgagttcccaggattctcgcgcttcaaggaacatcaaccctatggcgccccatctccgaaacggatatcagtaccacgatcgcacgccaagcatcccacagacacttatccagacgcatccgaagtcagcatcaaaaaagcaatcgcgacgtttctccctcgatttcaggacaaggagctcttcaatcgcgccttgtgctggtgtacagacactgcggacgctgctctcttgatgtgtgaacaccccaaatggaagaatttcattctagcgaccggcgacagcggacactcattcaaaatcttgcctaacgtcggaaaatacgtagtcgagttgatagagggccgcctgccggaggaaatggcttatcaatggaggtggcggccaggaggcgatgcactcaagtctagacgtgcggcaccgccaaaagatcttgcagacatgccaggatggaaacatgatccgaaattgtaa

SEQ ID NO: 3 - DNA, 30 bp, Artificial
  primer
tcatgggaatagcactgcgcaacaaggtgg

SEQ ID NO: 4 - DNA, 29 bp, Artificial
  primer
tattcccatgatcttgttgagatcatggc

SEQ ID NO: 5 - DNA, 29 bp, Artificial
  primer
acctgaaaaagctgtaccaggcactgcac

SEQ ID NO: 6 - DNA, 29 bp, Artificial
  primer
acctgaaaaagttctaccaggcactgcac

SEQ ID NO: 7 - DNA, 29 bp, Artificial
  primer
acctgaaaaagtattaccaggcactgcac

SEQ ID NO: 8 - DNA, 28 bp, Artificial
  primer
ctttttcaggtcctcgataccctcaggc

SEQ ID NO: 9 - DNA, 30 bp, Artificial
  primer
tcatgggaataaacctgcgcaacaaggtgg

SEQ ID NO: 10 - DNA, 30 bp, Artificial
  primer
tcatgggaatagatctgcgcaacaaggtgg

SEQ ID NO: 11 - DNA, 30 bp, Artificial
  primer
tcatgggaatacaactgcgcaacaaggtgg

SEQ ID NO: 12 - DNA, 30 bp, Artificial
  primer
tcatgggaatagaactgcgcaacaaggtgg

SEQ ID NO: 13 - DNA, 30 bp, Artificial
  primer
tgggaatagatctggccaacaaggtggacc

SEQ ID NO: 14 - DNA, 30 bp, Artificial
  primer
tgggaatagatctggaaaacaaggtggacc

SEQ ID NO: 15 - DNA, 30 bp, Artificial
  primer
tgggaatagatctgcacaacaaggtggacc

SEQ ID NO: 16 - DNA, 27 bp, Artificial
  primer
cagatctattcccatgatcttgttgag

SEQ ID NO: 17 - DNA, 28 bp, Artificial
  primer
tgagggtatcgaggccctgaaaaagctg

SEQ ID NO: 18 - DNA, 28 bp, Artificial
  primer
tgagggtatcgagaaactgaaaaagctg

SEQ ID NO: 19 - DNA, 28 bp, Artificial
  primer
tgagggtatcgagcgcctgaaaaagctg

SEQ ID NO: 20 - DNA, 28 bp, Artificial
  primer
ctcgataccctcaggcgtgtgttcgcag

SEQ ID NO: 21 - DNA, 30 bp, Artificial
  primer
aaaaagctgtaccagaaactgcacgatgcc

SEQ ID NO: 22 - DNA, 30 bp, Artificial
  primer
gcatcgtgcagtttctggtacagctttttc

SEQ ID NO: 23 - DNA, 30 bp, Artificial
  primer
aaaaagctgtaccagcgtctgcacgatgcc

SEQ ID NO: 24 - DNA, 30 bp, Artificial
  primer
gcatcgtgcagacgctggtacagctttttc

SEQ ID NO: 25 - DNA, 30 bp, Artificial
  primer
tcatgggaatagatgcgcgcaacaaggtgg

SEQ ID NO: 26 - DNA, 30 bp, Artificial
  primer
tcatgggaatagatgaccgcaacaaggtgg

SEQ ID NO: 27 - DNA, 30 bp, Artificial
  primer
tcatgggaatagatcatcgcaacaaggtgg

SEQ ID NO: 28 - DNA, 30 bp, Artificial
  primer
tcatgggaatagataagcgcaacaaggtgg

SEQ ID NO: 29 - DNA, 29 bp, Artificial
  primer
atctattcccatgatcttgttgagatcat

SEQ ID NO: 30 - DNA, 25 bp, Artificial
  primer
aggcgtgtgttcgcagtccattctg

SEQ ID NO: 31 - DNA, 30 bp, Artificial
  primer
gcgaacacacgcctaagggtatcgagaaac

SEQ ID NO: 32 - DNA, 29 bp, Artificial
  primer
acgtctagacttgagtgcatcgcctcctg

SEQ ID NO: 33 - DNA, 30 bp, Artificial
  primer
tcaagtctagacgtaaggcaccgccaaaag

SEQ ID NO: 34 - DNA, 30 bp, Artificial
  primer
acagacactgcggactctgctctcttgatg

SEQ ID NO: 35 - DNA, 28 bp, Artificial
  primer
gtccgcagtgtctgtacaccagcacaag

SEQ ID NO: 36 - protein, 436 aa, Aspergillus oryzae
MTVTKSSSILIIGAGTWGASTALHLGRRGYTNVTVLDPYTVPSAISAGNDVNKIISSGQYSNKKDEIEVNEILAEEAFKGWTTDPLFKPYYHDTGVVMSACSSAGLDRLGIRVRPEEEPDVSEVTKPEHFRQLAPAVLKGNFPGWRGYHIRSNAGWAHARNALVAAIREAEKLGVKFVTGTQGRVITLIFENNDVKGAVTADGKIWRAEQTVLCAGANAAQFLDFKDQLRPTAWTLAHIRLKPEERALYKNLPVIFNIEKGFFFEPDEERGEIKICDEHPGYTNMVKSADGHLTSLPFEKTQIPKESEARVRALLSETMPQLADRPFSFARVCWCADTANREFIIDRHPEHPSLVLGCGASGRGFKYLPSIGNLIVDAIEDKVPEKVHKLTRWSPDIAVDRKWRDTLGRFGGPNRVMDFHDVKEWTNVQNKDTAKL

SEQ ID NO: 37 - DNA, 1311 bp, Aspergillus oryzae
atgactgtcaccaaatcttcctcaatcctgatcatcggcgcaggcacttggggcgcttcaactgcccttcaccttggtcgcagaggatacaccaatgtcaccgtcctagacccttacacagtgccctcagcaatttcagctggaaatgacgtgaacaagatcatctcctcggggcaatacagcaacaaaaaggatgagattgaagttaacgaaattctcgccgaggaggcattcaaaggctggacaaccgaccctttgttcaagccatactaccacgacactggcgttgtaatgtctgcttgcagcagcgccggtctggatcgcctcggaatccgagtaaggccggaagaggaacctgatgtttccgaagtcacgaagccggagcacttccgccaactggcccccgctgtgctgaaaggaaacttcccggggtggagaggctaccacattcgttcgaacgctggctgggcgcacgcccgaaatgccctcgtggccgctatacgcgaagcagagaaacttggtgttaaattcgtaacaggcacccaaggaagagtcatcacccttatcttcgagaacaacgacgtcaagggcgcagtcaccgccgacggaaagatctggcgcgcggagcaaacagttctctgcgctggcgcaaatgctgcgcagttcttggattttaaggaccagctccgcccaacggcatggacactcgcccatatccggctcaaacctgaggaacgcgcgctctacaaaaacttgccggtgattttcaacattgagaaaggatttttcttcgagcctgatgaggagcgcggggagatcaagatctgcgacgaacatccgggatacactaacatggttaaatctgcggatggccacttgacgagtttgccctttgagaagacccagatccccaaggagtctgaagctagagtcagagctttactatcggagaccatgcctcaattagccgatcgcccatttagcttcgcccgcgtttgctggtgtgcggacaccgcaaaccgtgaattcatcattgaccgccaccctgaacacccgtctcttgttttgggatgcggtgcttccggaaggggtttcaaatatctcccctcaatcggcaacctcattgttgacgccattgaagacaaagtcccagagaaagttcacaagcttacgaggtggagtccagacattgctgttgacagaaagtggagggacactctggggcgctttggagggcctaaccgtgtcatggacttccatgatgtcaaggaatggactaacgtgcagaacaaggatactgcgaagctgtag

SEQ ID NO: 38 - protein, 437 aa, Phaeosphaeria nodorum
MAPSRANTSVIVVGGGGTIGSSTALHLVRSGYTPSNVTVLDAYPIPSSQSAGNDLNKIMGVSLRNPVDLQLALEARQMWNEDELFKKFFHNTGRLDCAHGEKDIADLKSGYQALVDAGLDATNEWLDSEDEILKRMPLLSRDQIKGWKAIFSKDGGWLAAAKAINAVGEYLRDQGVRFGFYGAGSFKAPLLAEGVCIGVETVDGTRYYADKVVLAAGAWSPTLVELHEQCVSKAWVYGHIQLTPEEAARYKNSPVVYNGDVGFFFEPNEHGVIKVCDEFPGFTRFKMHQPFGAKAPKRISVPRSHAKHPTDTIPDASDVSIRRAIATFMPQFKNKKMFNQAMCWCTDTADAALLICEHPEWKNFVLATGDSGHSFKLLPNIGKHVVELLEGTLADDLAHAWRWRPGSGDALKSRRSAPAKDLADMPGWNHDKPRANL

SEQ ID NO: 39 - DNA, 1314 bp, Phaeosphaeria nodorum
atggccccgtcgcgtgctaatacgtcggtcattgtggttggtggtggtggtacgattggctcatctacggctctgcatctggtccgctcaggctataccccgtcgaacgtgacggttctggatgcatacccgattccgagctctcagagcgctggcaacgacctgaataaaatcatgggtgtctctctgcgtaatccggtggatctgcagctggctctggaagcgcgccaaatgtggaacgaagacgaactgttcaagaagtttttccataacaccggccgtctggattgcgcgcacggtgaaaaagatattgccgacctgaagagcggctatcaggctctggtggatgcgggtctggacgccacgaacgaatggctggatagtgaagacgaaatcctgaaacgtatgccgctgctgtcccgcgatcaaattaaaggctggaaggcgatcttttcaaaagacggtggttggctggcagcagcaaaggcaattaatgcagttggtgaatatctgcgtgatcagggcgtccgcttcggtttttacggcgccggttctttcaaagcaccgctgctggctgaaggcgtctgcatcggtgtcgaaaccgtggatggcacgcgctattacgcagacaaagtggttctggctgcaggtgcatggtcgccgaccctggttgaactgcatgaacagtgtgtgagcaaagcgtgggtttacggccacattcaactgacgccggaagaagccgcacgttataagaacagcccggtcgtgtacaatggcgatgtgggctttttctttgaaccgaacgaacatggcgttatcaaagtctgcgatgaatttccgggttttacccgcttcaagatgcaccagccgtttggtgccaaagcaccgaagcgtattagtgtgccgcgctcccatgccaaacacccgaccgatacgatcccggatgcaagtgacgtttccattcgtcgcgctatcgcgacctttatgccgcagttcaagaacaaaaagatgttcaaccaagcgatgtgctggtgtaccgatacggccgacgctgcgctgctgatttgtgaacatccggaatggaaaaactttgttctggcgaccggcgattcaggtcattcgttcaaactgctgccgaatatcggcaagcacgttgtcgaactgctggagggtacgctggcagatgacctggcacacgcatggcgttggcgtccgggtagtggtgatgcactgaaaagccgtcgctctgctccggcgaaagacctggctgatatgccgggctggaaccatgacaaaccgcgtgctaatctgtaa

SEQ ID NO: 40 - protein, 437 aa, Eupenicillium terrenum
MAHSRASTKVVVVGGGGTIGSSTALHLIRSGYTPSNITVLDVYKTPSLQSAGHDLNKIMGIRLRNGPDLQLSLESLDMWQNDELFKPFFHQVGMIDCSSSKEGIENLRRKYQTLLDAGIGLEKTNVWLESEDEILAKAPNFTREQVKGWKGLFCTDGGWLAAAKAINAIGIFLQDKGVKFGFGDAGTFQQPLFAADGKTCIGLETTDGTKYFADKVVLAAGAWSPTLVDLEDQCVSKAWVFAHIQLTPKEADAYKNVPVVYDGEYGFFFEPDEYGVIKVCDEFPGFSRFKLHQPYGAASPKMISVPRSHAKHPTDTYPDASEVTIRKAIARFLPEFKDKELFNRTMCWCTDTADANLLICEHPKWKNFILATGDSGHSFKLLPNIGKYVVELLEGSLSQEMAGAWRWRPGGDALRSRRGAPAKDLAEMPGWKHDAHL

SEQ ID NO: 41 - DNA, 1314 bp, Eupenicillium terrenum
atggctcattcgcgtgcaagcaccaaagtcgtcgtggttgggggaggtggtacgatcgggtcttcgacggctctgcacttaatccgctctggatataccccctcaaatatcaccgtgcttgacgtatacaagaccccttcattgcaatctgcaggacatgatttgaacaagatcatgggcattcgattgcgcaacgggcctgacttgcagctttcgctggaatcactcgacatgtggcaaaacgatgagttgttcaagccattctttcaccaagtgggcatgattgattgttcgtcatccaaagagggtattgaaaatcttcgacgaaaataccagaccctcctcgatgcgggcattgggctggagaagacgaacgtttggctggaatctgaagatgagatcctcgccaaagcgccgaatttcacgcgtgaacaagtcaaggggtggaaaggcttattttgcactgatggaggctggcttgctgcagccaaggctatcaatgcgatcggaattttcctccaggacaaaggtgtcaagtttggctttggagatgctggtacctttcagcaacctctgttcgccgctgatggaaaaacttgcatcggacttgaaactacagacggaaccaagtactttgctgacaaggttgtcttggctgctggtgcgtggagtcccaccttggtggatctagaagatcagtgtgtttcaaaggcctgggttttcgctcatattcaactcacacccaaagaagcggacgcgtacaagaatgtgcctgtggtctatgatggtgaatatgggttctttttcgaacccgacgagtatggggtgatcaaagtctgtgacgagttccctggtttctctcgcttcaaactgcatcaaccgtacggggctgcatctcccaagatgatatccgtaccgcgatcacacgccaagcatcccacagatacctaccctgatgcctccgaagtcaccatacgcaaagcgatcgcaaggttcctgccagaatttaaagacaaggagctcttcaaccgtaccatgtgctggtgtacagatacggccgatgctaacttattgatttgcgaacacccgaagtggaagaatttcattctggccactggagatagcggacattccttcaagctgttgccaaacatcgggaaatacgtagttgagcttttagagggatctctatcgcaggaaatggctggtgcctggagatggagacccggaggtgatgctcttagatctagacgcggtgctccggcaaaggatcttgctgagatgccgggatggaagcatgatgcacatttgtga

SEQ ID NO: 42 - DNA, 30 bp, Artificial
  primer
aagatcatgggcattgatttgcgcaacggg

SEQ ID NO: 43 - DNA, 30 bp, Artificial
  primer
aatgcccatgatcttgttcaaatcatgtcc

SEQ ID NO: 44 - DNA, 30 bp, Artificial
  primer
gagggtattgaaaaacttcgacgaaaatac

SEQ ID NO: 45 - DNA, 26 bp, Artificial
  primer
ttcaataccctctttggatgacgaac

SEQ ID NO: 46 - DNA, 30 bp, Artificial
  primer
aaaaacttcgacgattataccagaccctcc

SEQ ID NO: 47 - DNA, 29 bp, Artificial
  primer
tcgtcgaagtttttcaataccctctttgg

SEQ ID NO: 48 - DNA, 30 bp, Artificial
  primer
cgacgattataccagaaactcctcgatgcg

SEQ ID NO: 49 - DNA, 30 bp, Artificial
  primer
ctggtataatcgtcgaagtttttcaatacc

SEQ ID NO: 50 - DNA, 30 bp, Artificial
  primer
agatacggccgattctaacttattgatttg

SEQ ID NO: 51 - DNA, 29 bp, Artificial
  primer
atcggccgtatctgtacaccagcacatgg

SEQ ID NO: 52 - DNA, 30 bp, Artificial
  primer
tcatgggcattgatcatcgcaacgggcctg

SEQ ID NO: 53 - DNA, 29 bp, Artificial
  primer
atcaatgcccatgatcttgttcaaatcat

SEQ ID NO: 54 - protein, 441 aa, Neocosmospora vasinfecta
MTTPRKETTVLIIGGGGTIGSSTALHLLRAGYTPSNITVLDTYPIPSAQSAGNDLNKIMGIRLRNKVDLQLSLEARDMWRNDALFRPFFHNTGRLDCESSAEGVEGLRREYQKLVEAGVGLEETHEWLDSEEAILEKAPLLQREEIEGWKAIWSEEGGWLAAAKAINAIGEELQRQGVRFGFGGAGSFKRPLFADDGTTCIGVETVDGTQYHADKVVLAAGAWSPALVDLEEQCCSKAWVYAHMQLTPEEAAVYKGCPVVYHGDVGFFFEPNENGVIKVCDEFPGFTRFKQHQPYGAPAPKPVSVPRSHAKHPTDTYPDASEESIKRAVSTFLPRFKDKPLFNRALCWCTDTADSALLICEHPRWKNFILATGDSGHSFKLLPIIGKHVVELVEGRLADDLAEAWRWRPGQGDARKSIRAAPAKDLADMPGWKHDQDSESR

SEQ ID NO: 55 - DNA, 1326 bp, Neocosmospora vasinfecta
atgacgaccccgcgtaaagaaacgacggtcctgattattggtggtggtggcacgattggtagctcgacggctctgcatctgctgcgtgccggctataccccgtctaacattaccgtgctggatacgtacccgatcccgagtgcccagtccgcaggcaacgacctgaataaaattatgggtatccgtctgcgcaataaagttgatctgcaactgagcctggaagcccgtgatatgtggcgcaacgacgcactgtttcgtccgtttttccataataccggccgcctggactgcgaaagctctgctgaaggcgtggaaggtctgcgtcgcgaatatcagaaactggtggaagcaggcgttggtctggaagaaacgcacgaatggctggatagcgaagaagctattctggaaaaagcgccgctgctgcaacgtgaagaaattgaaggttggaaagccatctggtctgaagaaggcggttggctggcggccgcaaaagctattaacgcgatcggcgaagaactgcagcgtcaaggcgttcgcttcggttttggcggtgccggtagttttaaacgcccgctgttcgcagatgacggcaccacgtgtatcggtgtcgaaaccgtggatggcacgcagtatcatgcggacaaagtggttctggctgcaggtgcttggtcaccggcgctggtcgatctggaagaacagtgctgttcgaaagcctgggtgtacgcacacatgcaactgaccccggaagaagccgcagtttataaaggctgcccggtcgtgtaccacggcgatgtcggctttttctttgaaccgaacgaaaatggcgttattaaagtctgtgacgaattcccgggttttacgcgtttcaaacagcatcaaccgtatggtgccccggcaccgaaacctgtgagtgttccgcgctcccatgcgaaacacccgaccgatacgtacccggacgcttcagaagaatcgatcaaacgtgccgtgagtacctttctgccgcgcttcaaagataaaccgctgtttaaccgtgcactgtgctggtgtaccgatacggccgactccgcactgctgatttgcgaacacccgcgctggaaaaattttatcctggcgaccggcgatagcggtcattctttcaaactgctgccgattatcggcaaacacgttgtcgaactggttgaaggtcgtctggcggatgacctggctgaagcgtggcgttggcgtccgggtcagggtgatgcacgtaaaagcattcgcgctgcgccggcgaaagacctggcggatatgccgggctggaaacacgaccaagactcggaatcacgctga

SEQ ID NO: 56 - DNA, 29 bp, Artificial
  primer
ttatgggtatcgatctgcgcaataaagtt

SEQ ID NO: 57 - DNA, 30 bp, Artificial
  primer
gctcagttgcagatcaactttattgcgcag

SEQ ID NO: 58 - DNA, 30 bp, Artificial
  primer
gaaggcgtggaaaaactgcgtcgcgaatat

SEQ ID NO: 59 - DNA, 30 bp, Artificial
  primer
ttccaccagtttctgatattcgcgacgcag

SEQ ID NO: 60 - DNA, 27 bp, Artificial
  primer
ctgcgtcgcctgtatcagaaactggtg

SEQ ID NO: 61 - DNA, 30 bp, Artificial
  primer
accaacgcctgcttccaccagtttctgata

SEQ ID NO: 62 - protein, 438 aa, Aspergillus nidulans
MTPRANTKIIVVGGGGTMGSSTALHLLRAGYTPSNITVLDTCPIPSAQSAGYDLNKIMGIRLRNKPDLQLSLEALDMWKNDPLFKPFFHNVGMIDVSSTEEGIEGLRKKYQSLLDAGIGLEKTNFMLESEDEILAKAPHFTQEQIKGWKGLFCGDGGWLAAAKAINAIGQFLKEQGVKFGFGGAGTFKKPLFADAHEKTCIGVETVDGTKYYADKVVLAAGAWSSTLVDLEEQCVSKAWVFAHIQLTPAEAAAYKNTPVIYDGDYGFFFEPNENGIIKVCDEFPGFTHFKMHQPYGSPAPKPISVPRSHAKHPTDTYPHASEVTIKKAINRFLPRFNDKELFNRAMCWCTDTADANLLVCEHPRWKGFYLATGDSGHSFKLLPNIGKHVVELLEERLESVFKDAWRWRPGSGDALKSRRAAPAKDLADMPGWRNEAKM

SEQ ID NO: 63 - DNA, 1317 bp, Aspergillus nidulans
atgacgccccgagccaacaccaaaatcattgtcgtcggcggcggcggcacaatgggctcgtcgacagccctacacctcctgcgcgccggctacacgccgtccaacattacagtgctcgacacgtgccctatcccctccgcacagtctgcaggctacgacctgaacaaaatcatggggatccgtctgcgcaacaagcctgatttacagctctctcttgaggcgctggacatgtggaaaaatgatcctctcttcaagccgtttttccacaatgttggaatgatcgacgtctcttcaacagaggaaggcatcgagggtcttcggaagaaataccagtctcttctcgacgcaggcattgggctcgagaagacgaatttcatgctggaaagtgaagacgagatcctggctaaagcgccgcatttcacgcaggagcagattaaaggctggaaaggcctgttctgtggcgacggcggctggctcgctgcagccaaagccatcaatgccattgggcagttcctcaaggaacagggcgtcaagtttggattcggcggcgccggcacgttcaaaaagccactcttcgccgatgcccacgagaagacgtgcatcggcgtcgagactgtagacggcacaaagtactacgccgacaaggtcgttctagcagctggtgcctggagttcgacgttggtcgatctggaggagcagtgcgtttcaaaggcctgggtctttgcccacatccaactgacgcccgctgaagcagccgcgtataagaacactcctgttatatacgacggtgactatgggtttttctttgagccgaatgaaaacggcatcataaaagtctgtgacgaattccctggcttcacgcatttcaaaatgcaccagccgtacggctcgccggcgcccaaacccatctctgtgcctcgttcccatgcgaagcaccccacagatacatacccgcacgcgtcggaggtcacgatcaaaaaggctatcaaccggttcctgccgaggttcaatgacaaggaactgtttaacagggccatgtgctggtgcaccgataccgcggatgcaaatctgcttgtttgtgagcatccacgctggaaggggttttatcttgcaacaggggacagtgggcattcgttcaagttgctgccgaatattggaaagcatgttgtcgagttattggaggagaggctggaaagtgtgtttaaggatgcttggaggtggaggcctggcagtggggatgcattaaaaagtagacgggctgcgcctgcgaaggacctggcggatatgccggggtggaggaatgaggcaaagatgtag

SEQ ID NO: 64 - DNA, 30 bp, Artificial
  primer
atcatgggcatcgatctgcgcaacaagcct

SEQ ID NO: 65 - DNA, 30 bp, Artificial
  primer
agagagctgtaaatcaggcttgttgcgcag

SEQ ID NO: 66 - DNA, 30 bp, Artificial
  primer
gaaggcatcgagaaacttcggaagaaatac

SEQ ID NO: 67 - DNA, 30 bp, Artificial
  primer
gtcgagaagagactggtatttcttccgaag

SEQ ID NO: 68 - DNA, 27 bp, Artificial
  primer
cttcggaagctgtaccagtctcttctc

SEQ ID NO: 69 - DNA, 30 bp, Artificial
  primer
cccaatgcctgcgtcgagaagagactggta

SEQ ID NO: 70 - DNA, 30 bp, Artificial
  primer
cttctcgagcccaatgcctgcgtcgagaag

SEQ ID NO: 71 - DNA, 30 bp, Artificial
  primer
gataccgcggatagcaatctgcttgtttgt

SEQ ID NO: 72 - DNA, 30 bp, Artificial
  primer
ccagcgtggatgctcacaaacaagcagatt

SEQ ID NO: 73 - DNA, 30 bp, Artificial
  primer
atcatgggcatcgatcatcgcaacaagcct

SEQ ID NO: 74 - DNA, 27 bp, Artificial
  primer
agagagctgtaaatcaggcttgttgcg

SEQ ID NO: 75 - DNA, 30 bp, Artificial
  primer
tcttcaacagagaaaggcatcgagaaactt

SEQ ID NO: 76 - DNA, 27 bp, Artificial
  primer
gtacagcttccgaagtttctcgatgcc

SEQ ID NO: 77 - DNA, 29 bp, Artificial
  primer
atcatgggtgtcgatctgcgtaatccggt

SEQ ID NO: 78 - DNA, 30 bp, Artificial
  primer
agccagctgcagatccaccggattacgcag

SEQ ID NO: 79 - DNA, 30 bp, Artificial
  primer
aaagatattgccaaactgaagagcggctat

SEQ ID NO: 80 - DNA, 30 bp, Artificial
  primer
atccaccagagcctgatagccgctcttcag

SEQ ID NO: 81 - DNA, 27 bp, Artificial
  primer
ctgaagagcctgtatcaggctctggtg

SEQ ID NO: 82 - DNA, 30 bp, Artificial
  primer
gtccagacccgcatccaccagagcctgata

SEQ ID NO: 83 - DNA, 30 bp, Artificial
  primer
agcctgtatcagaaactggtggatgcgggt

SEQ ID NO: 84 - DNA, 30 bp, Artificial
  primer
gttcgtggcgtccagacccgcatccaccag

SEQ ID NO: 85 - DNA, 30 bp, Artificial
  primer
gatacggccgacagcgcgctgctgatttgt

SEQ ID NO: 86 - DNA, 30 bp, Artificial
  primer
ccattccggatgttcacaaatcagcagcgc

SEQ ID NO: 87 - DNA, 29 bp, Artificial
  primer
atgggtgtcgatcatcgtaatccggtgga

SEQ ID NO: 88 - DNA, 30 bp, Artificial
  primer
cagagccagctgcagatccaccggattacg

SEQ ID NO: 89 - protein, 443 aa, Cryptococcus neoformans
MPPSRASTKVIVIGGGGTLGSSTALHLLRAGYTPSNITVLDTYLIPSAQSAGNDLNKIMGIRIRNPVDKQLSLEARDMWRNDEVFKPYFHNTGRLDCAHTPESIASLRKSYEAILKAGSGLEKTHHWLSTEDEILARAPLLDRKQIKGWKAIYSEDGGWLAAAKAINSIGQVLKEKGVTFGFGSAGSFKKPLFDEDGTKAIGIETVDGTQYFADKVVLAAGAWSPTLVDLEGQCCSKAWVYAHMQLTPEEAAEYKECPVVYNSELGFFFEPNEKGVIKVCDEFPGFTRFKQHQPYGASSTKHISFPRSHAKHPTDTIPDESDASIRRAISAFLPRFKEKELFNRALCWCTDTADANLLICEHPKWKNFILATGDSGHSFKILPNIGKHVVELIEGTLAEDLAESWRWRPGSGDPLISRRAAPARDLADLPGWNHDEPSDDDMD

SEQ ID NO: 90 - DNA, 1332 bp, Cryptococcus neoformans
atgccgccgtcccgtgcttcaacgaaagtgattgtcattggtggtggtggtacgctgggctcctcaaccgccctgcatctgctgcgcgcgggctataccccgagtaacattaccgtgctggatacgtacctgatcccgagtgcccagtccgcaggcaacgacctgaataaaattatgggtattcgtatccgcaatccggtggataaacaactgagcctggaagcccgtgatatgtggcgcaacgacgaagttttcaaaccgtacttccataacaccggtcgtctggactgcgctcacacgccggaatcaattgcgtcgctgcgtaaaagctacgaagccatcctgaaagcaggctcaggtctggaaaaaacccatcactggctgtcgacggaagatgaaatcctggcacgtgcaccgctgctggaccgtaaacagattaaaggttggaaagcaatctatagtgaagatggcggttggctggcggccgcaaaagctattaactccatcggccaagtcctgaaagaaaaaggtgtgaccttcggctttggtagcgcaggctcttttaaaaaaccgctgttcgatgaagacggcacgaaagccattggtatcgaaaccgttgatggtacgcagtattttgccgacaaagtggttctggctgcaggtgcatggagcccgaccctggttgatctggaaggccagtgctgttctaaagcttgggtctacgcgcacatgcaactgacgccggaagaagccgcagaatataaagaatgcccggtcgtgtacaacagcgaactgggctttttctttgaaccgaacgaaaaaggtgtgatcaaagtttgtgatgaattcccgggctttacccgtttcaaacagcatcaaccgtacggtgctagctctacgaaacacattagctttccgcgctctcatgcgaaacacccgaccgatacgatcccggatgaaagtgacgcctccattcgtcgcgctatctctgcgtttctgccgcgtttcaaagaaaaagaactgtttaaccgcgcgctgtgctggtgtaccgatacggctgacgcgaacctgctgatttgtgaacacccgaaatggaaaaattttatcctggccaccggcgattcaggtcattcgttcaaaattctgccgaatatcggcaaacacgttgtcgaactgattgaaggtaccctggccgaagatctggcagaaagctggcgttggcgtccgggcagtggtgacccgctgatctcccgtcgcgctgcgccggcgcgcgacctggcggacctgccgggctggaaccacgacgaaccgagcgacgatgacatggactga

SEQ ID NO: 91 - DNA, 30 bp, Artificial
  primer
attatgggtattgatatccgcaatccggtg

SEQ ID NO: 92 - DNA, 30 bp, Artificial
  primer
gctcagttgtttatccaccggattgcggat

SEQ ID NO: 93 - DNA, 30 bp, Artificial
  primer
gaatcaattgcgaaactgcgtaaaagctac

SEQ ID NO: 94 - DNA, 30 bp, Artificial
  primer
tttcaggatggcttcgtagcttttacgcag

SEQ ID NO: 95 - DNA, 30 bp, Artificial
  primer
ctgcgtaaactgtacgaagccatcctgaaa

SEQ ID NO: 96 - DNA, 30 bp, Artificial
  primer
acctgagcctgctttcaggatggcttcgta

SEQ ID NO: 97 - DNA, 30 bp, Artificial
  primer
aaactgtacgaaaaaatcctgaaagcaggc

SEQ ID NO: 98 - DNA, 30 bp, Artificial
  primer
tttttccagacctgagcctgctttcaggat

SEQ ID NO: 99 - protein, 440 aa, Curvularia clavata
MAPSRANTSVIVVGGGGTIGSSTALHLVRSGYTPSNITVLDAYPIPSSQSAGNDLNKIMGIRLRNKVDLQLSLEARQMWREDDLFKEYFHNTGRLDCAHGEEGLADLRQAYQALLDANAGLEETTEWLDSEDEILKKMPLLSRDQIKGWKAVYSQDGGWLAAAKAINAIGEYLRAQGVKFGFGGAGSFKQPLLAEGVCIGVETVDGTRYYADKVVLAAGAWSPTLVELHEQCVSKAWVYGHIQLTPEEAAEYKNSPVVYNGDVGFFFEPNEHGVIKVCDEFPGFTRFKMHQPFGAKAPKRISVPRSHAKHPTDTIPDASEKSIRKAIATFLPKFTEKELFNRHLCWCTDTADAALLICEHPEWKNFVLATGDSGHSFKLLPNIGKHVVELLEGTLADDLAHAWRWRPGSGDALKSRRSAPAKDLADMPGWKHDDVVKSKL

SEQ ID NO: 100 - DNA, 1323 bp, Curvularia clavata
atggccccgtcgcgtgctaatacgtcggtcattgtggttggtggtggtggtacgattggctcatctacggctctgcatctggtccgctcaggctataccccgtcgaacattacggttctggatgcatacccgattccgagctctcagagcgctggcaacgacctgaataaaatcatgggtatccgtctgcgtaataaggtggatctgcagctgtctctggaagcgcgccaaatgtggcgcgaagacgatctgttcaaggagtatttccataacaccggccgtctggattgcgcgcacggtgaagaaggtcttgccgacctgcgtcaagcctatcaggctctgctggatgcgaatgcgggtctggaagagacgaccgaatggctggatagtgaagacgaaatcctgaaaaaaatgccgctgctgtcccgcgatcaaattaaaggctggaaggcggtgtattcacaggacggtggttggctggcagcagcaaaggcaattaatgcaattggtgaatatctgcgtgctcagggcgtcaaattcggttttggcggcgccggttctttcaaacaaccgctgctggctgaaggcgtctgcatcggtgtcgaaaccgtggatggcacgcgctattacgcagacaaagtggttctggctgcaggtgcatggtcgccgaccctggttgaactgcatgaacagtgtgtgagcaaagcgtgggtttacggccacattcaactgacgccggaagaagccgcagaatataagaacagcccggtcgtgtacaatggcgatgtgggctttttctttgaaccgaacgaacatggcgttatcaaagtctgcgatgaatttccgggttttacccgcttcaagatgcaccagccgtttggtgccaaagcaccgaagcgtattagtgtgccgcgctcccatgccaaacacccgaccgatacgatcccggatgcaagtgaaaaatccattcgtaaagctatcgcgacctttctgccgaagttcacggagaaagagctgttcaaccgtcatctgtgctggtgtaccgatacggccgacgctgcgctgctgatttgtgaacatccggaatggaaaaactttgttctggcgaccggcgattcaggtcattcgttcaaactgctgccgaatatcggcaagcacgttgtcgaactgctggagggtacgctggcagatgacctggcacacgcatggcgttggcgtccgggtagtggtgatgcactgaaaagccgtcgctctgctccggcgaaagacctggctgatatgccgggctggaaacatgacgatgtggtgaaaagcaaactgtaa

SEQ ID NO: 101 - DNA, 30 bp, Artificial
  primer
atcatgggtatcgatctgcgtaataaggtg

SEQ ID NO: 102 - DNA, 30 bp, Artificial
  primer
cagagacagctgcagatccaccttattacg

SEQ ID NO: 103 - DNA, 30 bp, Artificial
  primer
gaaggtcttgccaaactgcgtcaagcctat

SEQ ID NO: 104 - DNA, 30 bp, Artificial
  primer
atccagcagagcctgataggcttgacgcag

SEQ ID NO: 105 - DNA, 30 bp, Artificial
  primer
cttgccaaactgcgtcaactgtatcaggct

SEQ ID NO: 106 - DNA, 30 bp, Artificial
  primer
acccgcattcgcatccagcagagcctgata

SEQ ID NO: 107 - DNA, 30 bp, Artificial
  primer
cgtcaactgtatcagaaactgctggatgcg

SEQ ID NO: 108 - DNA, 30 bp, Artificial
  primer
ctcttccagacccgcattcgcatccagcag

SEQ ID NO: 109 - DNA, 30 bp, Artificial; identical to SEQ ID NO: 85
  primer

SEQ ID NO: 110 - DNA, 30 bp, Artificial; identical to SEQ ID NO: 86
  primer

SEQ ID NO: 111 - DNA, 30 bp, Artificial
  primer
atcatgggtatcgatcatcgtaataaggtg

SEQ ID NO: 112 - DNA, 30 bp, Artificial
  primer
aagctgtaccagaaacttctcgacgcaggc

SEQ ID NO: 113 - protein, 440 aa, Pyrenochaeta sp.
MAASRAKTTVIVVGGGGTIGSSTALHLLRSGYTPSNITVLDTYPIPSLQSAGNDLNKIMGIRLRNKVDLQLSLEAREMWREDELFRDFFHNTGRLDCAHGEKGINDLRQAYQTLLDANAGLEETNEWLDSEDEILARMPLLSREQIKGWKAVFSRDGGWLAAGKAINAIGEYLRKEGVKFGFGGAGSFQQPLLAEGICIGVETTDGTRYYADKVVLAAGAWSPALVDLEDQCVSKAWVYAHMQLTPKEAAAYKDTPVVYNGDLGFFFEPNEHGVIKVCDEFPGFTRFKKHQPFGARAPKRISVPRSHAKHPTDTYPHASEASIKKAIAAFLPQFKDKELFNRAMCWCTDTADAALLICEHPQWKNFMLATGDSGHSFKLLPNIGKHVVELIEGTLAADLAHAWRWRPGIGDALQSRRAAPAKDLADMPGWNHDESPRAKL

SEQ ID NO: 114 - DNA, 1323 bp, Pyrenochaeta sp.
atggccgcttcacgagcaaagacgacagtgatcgtcgtgggtggcggcggtaccattgggtcatcaacagcgctccaccttctacgttcaggttatactccatcgaatatcacagttttggacacatatccaattccttcattacagtccgcgggcaatgatttaaacaagattatgggcattcgcttgcgaaacaaagtcgacctccaattgagtttagaggctagggagatgtggagagaagatgaactttttagagatttttttcacaatactgggcgactggattgtgcccatggcgaaaaaggaatcaatgatcttaggcaggcatatcaaacactactcgacgccaatgccggtttggaagagacgaacgagtggctggactctgaggacgaaattctggcaagaatgccgctcttgagtcgagagcagatcaagggctggaaagcggtcttcagccgagacggcggttggctcgccgcaggtaaggccatcaatgcaattggcgagtatctgcgcaaggaaggagtcaagtttggctttggcggcgcgggatcgttccagcagccgcttcttgcagagggtatttgcattggcgtggaaacaacggatggaactagatactacgccgacaaagttgtcctggcagctggtgcatggagtcctgcattggtggacttggaagaccagtgtgtttcaaaagcatgggtctatgctcacatgcagctcaccccgaaggaggctgcggcatacaaagacacaccagtagtctacaatggcgatctgggatttttctttgaaccaaacgagcatggcgtgatcaaagtctgcgacgagttcccaggcttcacacgttttaagaagcatcaaccatttggtgcaagggcaccaaaacggatatcggttcccagatctcatgccaaacaccctactgatacttatcctcacgcatccgaagccagtatcaagaaagctattgcggcattcttaccacagttcaaggacaaggagctgttcaaccgcgcaatgtgctggtgcacagatacagctgatgcagccttgttgatctgcgaacacccgcaatggaagaatttcatgcttgctactggagacagcgggcactcatttaagctcttaccaaatatcggcaagcatgtagttgaactgattgaaggcactctggcggcagatcttgcccatgcttggaggtggcgacctgggattggtgacgctttgcagtcaaggcgagcggcacctgcgaaggatctggcggacatgccaggatggaatcatgatgaatctcctagggcgaaattgtaa

SEQ ID NO: 115 - protein, 452 aa, Arthrinium sp.
MAASRKTTKVIVVGGGGTIGSSTALHLLRSGYTATNITVLDTYPIPSAQSAGNDLNKIMGIRLRNPVDKQLSLEAQDMWCHDELFKPYFHNTGRMDCEGTEKGIAALKQQYQTLLDADVGLEKTTEWLDSEDAILAKMPLLERDQIKGWKAIFSQDGGWLAAAKAINAIGEELKRQGVNFGFGGAGAFKKPLFAPDGSTCIGVETVDGTKYYGDKVVLAAGAWSPALVDLEEQCCSKAWVYAHMQLTPHEAAEYQGCPVVYHGDLGFFFEPNEHGVIKVCDEFPGFTRFLEQHQSYGAPAPTRVSVPRSHAKHPTDTYPDASEQSIRRAVAAFLPRFQSKELFNRAMCWCTDTADAALLICEHPRWRNFILATGDSGHSFKLLPNIGKHVVELLEGRLADDLAQAWRWRPGQGDALKSRRAAPAKDLADMPGWNHDGDSGNATSGTSSEHKL

SEQ ID NO: 116 - DNA, 1359 bp, Arthrinium sp.
atggcggcgtcacgaaagaccaccaaagtgattgtcgtgggcggcggaggcaccatcggctcatccacggctctacatcttctccggtcggggtatacggccaccaacattaccgtcctggacacctaccccatcccctcggcgcagtcggccggcaacgacctgaacaagattatggggatccgcctgcggaacccggtcgacaagcagctcagccttgaagcccaggacatgtggtgccatgacgagctcttcaagccctacttccacaacaccggcaggatggactgcgagggcaccgagaagggcatcgcggcgctcaagcagcagtaccagaccttgcttgacgccgacgtgggcctcgagaagacgacggagtggctcgacagtgaggatgccatcctggcaaagatgccactcctggagcgcgaccaaatcaaaggatggaaagcgatatttagccaggacggcggttggctggccgcagctaaagccatcaacgcgataggcgaggaactgaagaggcagggcgtcaacttcgggttcggcggggcgggcgccttcaagaagccccttttcgccccggacggatccacctgcatcggcgtcgagacggtggatggaaccaagtactacggcgacaaggtcgtcctggccgcgggcgcgtggagccctgcgctggtcgacctggaagagcagtgctgctccaaggcctgggtgtacgcccacatgcagctgacgccgcacgaggcagccgagtaccagggctgtccggtcgtgtaccacggcgacctcggcttcttcttcgagcccaacgagcacggcgtcatcaaggtgtgcgacgagttccccggcttcacgcggttcctcgagcagcaccagtcgtacggcgcgccggcgccgacgcgcgtctcggtgccccggtcgcacgcgaagcaccccaccgacacatacccggacgcgtcggagcagtcgatccggcgggccgtggccgcgttcctgccgcgattccaaagcaaagagcttttcaaccgcgccatgtgctggtgcaccgacacggccgacgccgcgctgctgatctgcgagcacccccgctggcgcaattttattctggctacgggcgacagcggacactcgttcaagctcctgcccaacatcggcaagcacgtggtcgagctgctggaaggccggctagcggatgacctggcgcaggcgtggaggtggcgccccggtcagggggatgcgttgaagtctagacgggcggctccggctaaggatctggcggatatgccagggtggaatcatgacggggattcagggaatgctacgtctggaacaagctcggagcacaaattgtag

SEQ ID NO: 117 - protein, 440 aa, Curvularia clavata
MAPSRANTSVIVVGGGGTIGSSTALHLVRSGYTPSNITVLDTYPIPSAQSAGNDLNKIMGIRLRNKVDLQLSLEARQMWREDDLFKEYFHNTGRLDCAHGEEGLADLRQAYQALLDANAGLEETTEWLDSEDEILKKMPLLDREQIKGWKAVYSQDGGWLAAAKAINAIGEYLRAQGVKFGFGGAGSFKQPLLAEGVCIGVETVDGTRYYADKVVLAAGAWSPVLVDLEDQCVSKAWVYAHIQLTPEEAAEYKNVPVVYNGDVGFFFEPDEHGVIKVCDEFPGFTRFKQHQPYGAKAPKRISVPRSAAKHPTDTYPDASEKSIRKAIATFLPKFTEKELFNRHLCWCTDTADAALLMCEHPEWKNFVLATGDSGHTFKLLPNIGKHVVELLEGTLAEDLAHAWRWRPGTGDALKSRRAAPAKDLADMPGWKHDDVVKSKL

SEQ ID NO: 118 - DNA, 1323 bp, Curvularia clavata
atggcgccctcaagagcaaacacttctgttatcgttgtcggtggcggtggcactattggctcttcaaccgctcttcatctagtccgctcgggctacacaccatctaacatcaccgttcttgacacataccctatcccatcagcgcagtcagctggaaatgacctgaataagatcatgggtatccgcttgcggaacaaggtcgatctccaattgagtctagaagccaggcagatgtggagagaggatgacctattcaaagagtatttccacaacactggaagactcgactgtgcacatggggaagagggacttgcagatttgagacaggcataccaggctctgctcgacgctaacgcgggtctcgaagaaacaacagaatggcttgactccgaagacgaaattctaaagaaaatgccgcttctggaccgcgagcaaatcaagggctggaaagcggtttacagccaagacggcggctggctggctgcagcaaaagccatcaatgctataggcgagtacttgcgagcccaaggagttaagtttggttttggtggtgctggatcgttcaagcagcctcttttggccgagggagtgtgcattggcgtagagacagtcgacgggacgaggtactacgccgataaagttgtgcttgcagctggtgcttggagtccggtattggtcgacctggaagatcaatgcgtttcaaaagcttgggtatatgctcacatacagcttacgcctgaggaagcagcagagtacaaaaacgtgcctgtggtatacaacggcgacgtcggcttcttcttcgagcctgacgagcacggcgttatcaaggtttgtgacgaatttccaggttttacacgcttcaagcaacatcagccatatggcgccaaagcaccgaaacgtatctccgtgcccagatcggcagcgaagcacccgacggatacttaccccgatgcgtcggagaagagcatccgcaaggccattgcaactttcctgcccaagttcacagagaaggagctattcaaccggcatctatgttggtgtacggatacggctgacgctgcgctattgatgtgtgagcatcccgagtggaagaactttgtgctggcgacaggggacagcgggcacacattcaaacttttgccaaatatcggcaagcatgtggttgagcttctcgagggtacactcgcggaggatctggcacatgcatggagatggcggcctggtactggcgatgcgctgaaatcaagaagagcggcaccggcgaaggatttagcagatatgcctggctggaagcatgacgatgttgtcaagtccaagttatag

SEQ ID NO: 119 - protein, 438 aa, Emericella nidulans
MAPRANTKIIVVGGGGTMGSSTALHLLRAGYTPSNITVLDTYPIPSAQSAGYDLNKIFGIRLRNKPDLQLYLEALDMWKNDPLFKPFFHNVGQMDVSSTEEGIKKLRMRYQSLLDAGIGLEKTNFLLESEDEILAKAPHFTREQIKGWKGLFCGDGGWLAAAKAINAIGQFLKEQGVKFGFGEAGTFKKPLFADADEKTCIGVETVDGTKYYADKVVLAAGAWSSTLVDLEEQCVSKAWVFAHIQLTPAEAAAYKNTPVIYDGDYGFFIEPDENGIIKVCDEFPGFTHFKMHQPYGSPVPKLISVPRSHAKHPTDTYPHASEVTIKKAINRFLPRFNDKELFNRAMCWCTDTADANLLVCEHPRWKGFYLATGDSGHSFKLLPNIGKHVVELLEGRLESVFKDAWRWRPGSGDALKSRRAAPAKDLADMPGWRNEAKM

SEQ ID NO: 120 - DNA, 1317 bp, Emericella nidulans
atggcgccccgagccaacaccaaaatcatcgtcgtcggcggcggcggcacaatgggctcgtcgacagccctacacctcctgcgcgccggctacacgccgtccaacatcacagtgctcgacacgtaccctatcccttccgcacagtctgcaggctacgacctgaacaaaatcttcggcatcaggctgcgcaacaagcctgacttacaactctatcttgaggcgctggacatgtggaaaaatgatcctctattcaagccgtttttccacaatgttggacagatggacgtctcttcaacagaagaaggcatcaaaaagcttcgcatgagataccagtctcttctcgacgcaggcattgggctcgagaagacgaatttcctgctggaaagtgaagacgagatcctggctaaagcgccgcatttcacgcgggagcagattaaaggctggaaagggctgttctgtggcgacggcggttggctcgctgcagccaaagccatcaatgccatcgggcagttcctcaaggaacagggcgtcaagtttggatttggcgaggccggcacgttcaaaaagccactcttcgccgatgccgacgagaagacgtgcatcggcgtcgaaactgtagacggcacaaaatactacgccgacaaggtcgttctagcagctggtgcctggagttcgacgttggtcgatctggaggagcagtgcgtttcaaaggcctgggtctttgcccacatccaactgacgcccgctgaagcagccgcgtacaagaacactcctgttatatacgacggtgactatgggtttttcattgagccggacgagaacggcatcataaaagtctgcgacgaattccctggcttcacgcacttcaagatgcaccagccgtacggctcaccggtgcccaaattgatctctgtgcctcgctcccatgcgaagcaccccacagatacatacccgcacgcgtcggaggtcaccatcaaaaaggctatcaaccggttcctgccgaggttcaatgacaaggaactgtttaacagggccatgtgctggtgcaccgataccgcggatgcaaatctgcttgtttgtgagcatccacgctggaaggggttttatcttgcaacaggggacagcgggcattcgttcaagttgctgccgaatattggaaagcacgttgtcgagttattggaggggaggctggaaagtgtgtttaaggatgcttggaggtggaggcctggcagtggggatgcattaaagagtagacgggctgcgcctgcgaaggacctggcggatatgccggggtggaggaatgaggcaaagatgtag

SEQ ID NO: 121 - protein, 441 aa, Ulocladium sp.
MAPNRANISVIVVGGGGTIGSSTALHLVRSGYTPSNITVLDTYPIPSAQSAGNDLNKIMGIRLRNKVDLQLSLEARQMWTEDDLFKEYFHKTGRLDCAHGEKGLADLKQAYQALLDANAGLEATTEWLDSEDKILEKMPLLNRDQIKGWKAVFSEDGGWLAAAKAINAIGRFLRDQGVKFGFGGAGSFKQPLLAEGVCVGVETVDGTRYYADKVVLAAGAWSPALVDLQDQCVSKAWVYAHIQLSPSEAAEYKNVPVVYNGDVGFFFEPDEYGVIKVCDEFPGFTRFKQHQPFGASAPKRISVPRSAAKHPTDTYPDASEVSIRKAIATFLPKFTEKEVFNRHLCWCTDTADAALLMCEHPEWKNFVLATGDSGHTFKLLPNIGKHVVELLEGTLADDLAHAWRWRPGTGDALKSRRAARAKDLADMPGWNHDGEAPRAKL

SEQ ID NO: 122 - DNA, 1326 bp, Ulocladium sp.
atggcacctaacagagctaatatttctgtcatcgtcgtgggtggtggcggcaccattgggtcttcaacggcccttcatctcgtacgctcgggatacacaccgtcgaatatcacggttctggacacttatccaattccatcagcgcaatcagctggcaatgacttgaacaagatcatgggtatccgtttgcggaacaaggtggatttgcagttgagcttagaggcgagacaaatgtggacagaagacgatctgttcaaggagtactttcataaaaccgggcggctcgactgcgcacatggcgagaaaggccttgcagatctcaaacaagcctaccaagcccttcttgatgcgaacgctggcctggaggcgacgacagaatggttagattccgaggacaagattcttgagaagatgccgcttctcaatcgcgatcagatcaaaggatggaaagccgtcttcagcgaagacggcggatggctcgctgcggcaaaagccatcaacgctatcggtagatttctgcgcgatcaaggcgtcaagtttggctttggcggagcaggatcattcaaacaacctcttcttgccgagggtgtttgtgttggtgttgaaacagttgacgggacgagatattatgctgacaaggttgtgttggcggctggtgcgtggagtcctgcattggtcgatctacaagaccaatgtgtgtcgaaagcatgggtatacgctcacatccaactgtccccgagcgaggcggcggaatacaaaaatgttcctgtagtctataatggcgacgtgggcttcttcttcgagcctgacgaatacggcgtcatcaaagtctgtgacgagtttccaggttttacgcgcttcaagcagcatcaacctttcggcgcatcggctccaaagcgcatttctgtgcctcgatctgccgcaaaacaccccacagatacctatccggacgcctcggaagtcagtatccgcaaggccatcgcgacgttcctgcccaagttcacagaaaaggaagtgttcaacaggcatctgtgttggtgtactgatacggctgatgcggcgcttttgatgtgcgaacatcctgagtggaagaactttgttttggccacgggtgacagtggtcacaccttcaagcttctacctaacatcggtaagcatgtggtcgagctactagagggtacattagcagacgacctagcgcatgcgtggagatggcgtcccggtaccggcgatgcgctgaagtcgcgaagggcggcgcgtgcgaaagaccttgcagatatgccaggatggaatcatgacggggaagcccccagagcgaagctgtga

SEQ ID NO: 123 - protein, 437 aa, Penicillium janthinellum
MAHSRESTKIVIVGGGGTMGSSTALHLIRSGYTPSNITVLDVYPIPSLQSAGYDLNKIMSIRLRNGPDLQLSLEALDMWKNDPLFKPFFHNVGMLDCSSSQEGIASLRRKHQDLIDANIGLEKTNIWLESEDDILAKAPHFTREQIKGWKGLFCGDGGWLAAAKAINAIGTFLKSQGVKFGFGSAGTFKRPLFAPDGATCSGVETVDGTKYFADKVVLAAGAWSSTLVDLEDQCVSKAWVFAHIQLTPQESAQYKDVPVVYDGDYGFFFEPNEHGVIKVCDEFPGFSRFKLHQPYGATSPKLISVPRSHAKHPTDTYPDSSEETIRKAIARFMPRFKDKELFNRSMCWCTDTADANLLICEHPKWKNFILATGDSGHSFKVLPNIGKHVVELIEGRLPQDLAGAWRWRPGGDALKSKRSAPAKDLAEMPGWKHDAKL

SEQ ID NO: 124 - DNA, 1314 bp, Penicillium janthinellum
atggctcattcgcgagaaagcacaaagattgtcattgtcgggggaggtggcacaatgggatcttcaaccgcgctacacctgatacgctctggatacaccccgtcaaacatcaccgtccttgatgtatacccaattccatccttgcaatccgcaggatatgatcttaacaagatcatgagcatccgattacgcaacgggcctgacttgcaactttccctggaggctctcgatatgtggaaaaacgatccgttgttcaagcctttctttcacaacgttggcatgctagactgttcatcgtcacaagagggtattgcaagccttcgacggaagcaccaagacctcatagacgcgaatatcggactagagaagacgaatatctggttagagagtgaagatgatattctggcaaaagccccgcacttcacgcgggaacagatcaaggggtggaagggcttgttttgcggcgatggaggatggcttgctgcagccaaggccatcaatgcgatcggaacctttctaaaaagtcaaggcgtcaagttcggatttggaagtgccgggactttcaagcgacctttgtttgctccagatggggcgacatgcagcggtgttgagacagtagatggaacaaaatacttcgccgacaaggtggttttggccgctggtgcttggagttcgacgttagtagatttggaggaccaatgtgtttcgaaggcctgggtcttcgctcatatccaactcacgccccaagaatcggcccagtacaaggacgtgcccgtagtatacgacggtgattatggctttttcttcgagcccaacgaacacggagtaatcaaagtctgcgatgagttccccgggttctcccgcttcaagctgcatcaaccttacggtgccacctctcctaagcttatatccgttcctcgatcacacgccaagcatcccaccgatacctacccagattcttctgaagagaccattcgaaaagcgattgcgaggtttatgccacgcttcaaggataaggagctttttaataggagcatgtgctggtgcaccgatactgctgatgccaacttgttgatctgcgagcaccccaagtggaagaactttatcttggccacaggagacagcggccatagtttcaaggttttgcccaatataggaaaacatgtcgttgagttgatagaaggacgcctaccacaagacctggctggtgcgtggagatggagaccagggggagatgcccttaagtccaaacgcagtgctccggcaaaggaccttgctgaaatgccgggctggaagcatgatgcgaagctctga

SEQ ID NO: 125 - protein, 445 aa, Aspergillus fumigatus
MAPSILSTESSIIVIGAGTWGCSTALHLARRGYKDVTVLDPHPVPSPIAAGNDINKIMEHSELKDGSSDPRSAAFSTFTRAALKAWKTDPVFQPYFHETGFIISGHTPALIDHIRKDEVEPSETNFVKLETAEDFRRTMPPGVLTGDFPGWKGWLHKSGAGWIHAKKAMISAFNEAKRLGVRFVTGSPEGNVVSLVYEDGDVVGARTADGRVHKAHRTILSAGAGSDSLLDFKKQLRPTAWTLCHIQMGPEEVKQYRNLPVLFNIAKGFFMEPDEDKHELKICDEHPGYCNFLPDPNRPGQEKSVPFAKHQIPLEAEARARDFLHDTMPHLADRPLSFARICWDADTPDRAFLIDRHPEHPSLLVAVGGSGNGAMQMPTIGGFIADALESKLQKEVKDIVRWRPETAVDRDWRATQNRFGGPDRIMDFQQVGEDQWTKIGESRGP

SEQ ID NO: 126 - DNA, 1338 bp, Aspergillus fumigatus
atggcgccttcaattttgagcactgaatcttccattatcgttatcggagcaggcacatggggctgctcaactgctctgcacctcgctcgtcgaggctacaaagatgtcactgttctcgaccctcatccagttccttcgcccattgcagcaggcaatgacatcaacaagattatggagcacagcgagctgaaagatggctcatccgaccctcgaagcgcagccttctcgacatttacgcgagctgctcttaaggcgtggaaaactgacccggttttccagccttactttcacgaaactggctttatcatatcggggcacacacctgctctgattgaccacatacgaaaagacgaggtagaaccgtcagaaacaaacttcgtcaagctggagacagccgaggacttccgccggaccatgccgccaggtgtactgacaggcgacttccctggctggaaaggctggttgcacaagtctggtgctgggtggattcatgccaaaaaggctatgatctctgctttcaatgaagctaagcgcttgggagtcagatttgtcactggctctccggaagggaatgttgtatcgttggtatacgaggacggagacgtcgttggagccagaactgccgatggtcgcgtgcacaaagcccatcgcactattctttcggcaggtgctggcagtgacagtctcctagacttcaagaagcagcttcggcctaccgcgtggactctctgtcatattcagatgggccctgaagaggtcaagcaatatcggaaccttcctgtgttgttcaacatcgccaaagggttcttcatggagcctgatgaggataaacacgagctcaagatttgtgacgagcatccagggtactgcaactttctccctgacccaaacagaccgggccaggagaagagtgtccccttcgcaaagcatcagatcccgctcgaggccgaagcccgcgcacgagactttctccatgatacaatgccgcatctggctgaccggccactgtctttcgcgcgtatttgctgggatgctgataccccagaccgtgctttcttgatcgatagacatcctgaacacccctcactgctagtcgctgttggaggttccggcaatggcgccatgcaaatgcctacaattggcggttttatcgcagatgctctagagagtaaactacagaaggaggtgaaggacatcgttcgatggaggccagagacggctgtcgatcgagattggagagcgactcagaatcgctttggcgggcctgacaggatcatggattttcagcaggtcggagaggatcagtggaccaagattggagagagcagaggtccgtaa

SEQ ID NO: 127 - protein, 445 aa, Aspergillus oryzae
MTSSKLTPTSSILIVGAGTWGCSTALHLARRGYKNVTVLDPHPVPSPIAAGNDINKIMEHREVKASETDPWSIAFSTCTRAALKGWKNDPVFQPYFHETGAIVSGHTASLIKHIQEHEIDSSDAEFIKLNTAEDFRKTMPPGILTGNFPGWKGWLNKTGAGWIHAKKAMFSAYTEAKRLGVTFITGSPEGDVVSLIYENGDVVGARTADGTVHRADHTILSAGAGSDRLLDFKKQLRPTAWTLCHIRMTPDEAKKYRNLPVLFNVAKGFFMEPDEDNHELKICDEHPGYCNFVPDPKHGGEVRSIPFAKHQIPLEAEARARDFLRDTMPHLADRPLSFARICWDADTVDRAFLIDRHPEYRSLLLAVGGSGNGAMQMPTIGGFIADALEGNLQKELKHALRWRPEIAAQRDWKDTQNRFGGPNKVMDFQKVGENEWTKIGDKSRL

SEQ ID NO: 128 - DNA, 1338 bp, Aspergillus oryzae
atgacatcctccaagttgactcccacatcatctatcttaattgtcggtgcagggacctggggttgttctactgctttacatcttgcccgtcgaggatacaaaaatgtcacggtcctagatccgcacccggtcccttctcccattgcagctggcaatgacattaacaagattatggagcacagggaggtaaaagcctctgaaaccgatccttggagtatcgccttctcaacatgcacacgagctgcactgaaaggttggaaaaacgacccagtattccagccatacttccatgaaacgggggcaatagtttctggccacaccgcctctttgattaaacatatacaagaacacgaaatcgactcgtcagacgccgagttcataaaattgaacaccgcagaggatttccgcaaaactatgcccccgggaatcctcactggcaacttccccggctggaagggctggctgaacaagaccggcgccggatggatccacgccaagaaggccatgttctccgcatacaccgaagcaaagcgcctaggagtcactttcatcaccggctcccctgaaggagacgttgtatctctaatttacgagaatggagacgtagtcggagccagaacggccgacggcaccgtccaccgagcagaccataccattctttccgcaggggctggcagtgatcgtctcctggactttaagaaacagctccgtcctaccgcctggacgctctgccacatcagaatgacgcccgacgaggccaagaagtaccggaatcttcctgtgctgttcaacgtcgctaaggggttcttcatggaacctgatgaggataatcatgagcttaagatctgcgacgagcatcctggatattgcaacttcgtcccggacccgaagcacggcggtgaggtgcgcagtatcccatttgcaaagcatcagattcctcttgaagccgaggcccgtgcaagggacttcctccgtgatacgatgcctcatcttgctgatcgaccactgtcttttgctcgtatatgctgggatgctgatacagtggatcgcgccttcttgatcgataggcatcctgagtatcgctctttactgcttgctgtcggtggatctggtaatggagccatgcaaatgcctaccattggtgggttcatagcggatgctctggagggaaacctgcaaaaggaactgaagcatgcactacggtggaggcctgagattgccgcccaacgagactggaaggatacgcaaaatagattcggaggtccgaataaagtaatggatttccaaaaggttggagagaatgagtggaccaagattggcgataagagtcggctttaa

SEQ ID NO: 129 - protein, 438 aa, Aspergillus fumigatus
MAVTKSSSLLIVGAGTWGTSTALHLARRGYTNVTVLDPYPVPSAISAGNDVNKVISSGQYSNNKDEIEVNEILAEEAFNGWKNDPLFKPYYHDTGLLMSACSQEGLDRLGVRVRPGEDPNLVELTRPEQFRKLAPEGVLQGDFPGWKGYFARSGAGWAHARNALVAAAREAQRMGVKFVTGTPQGRVVTLIFENNDVKGAVTGDGKIWRAERTFLCAGASAGQFLDFKNQLRPTAWTLVHIALKPEERALYKNIPVIFNIERGFFFEPDEERGEIKICDEHPGYTNMVQSADGTMMSIPFEKTQIPKEAETRVRALLKETMPQLADRPFSFARICWCADTANREFLIDRHPQYHSLVLGCGASGRGFKYLPSIGNLIVDAMEGKVPQKIHELIKWNPDIAANRNWRDTLGRFGGPNRVMDFHDVKEWTNVQYRDISKL

SEQ ID NO: 130 - DNA, 1317 bp, Aspergillus fumigatus
atggcggtaaccaagtcatcttcccttttgatcgtgggggcaggcacctggggcacatcgactgctctccacctggcacgaagaggatacacaaatgtgacggttctagatccctaccccgttccctcagccatctcggctgggaatgatgtgaacaaggtcatctcctccggccaatatagcaacaacaaggacgaaattgaggtcaacgagattctggctgaagaagcgttcaatggctggaagaacgaccccttgttcaaaccatactatcacgatactggattgctcatgtccgcctgctcccaggaaggcttggaccgccttggagtccgtgtcaggcccggtgaggaccccaaccttgtggaactgacacggccggagcaattccgcaaattagctcctgagggtgttctacagggagatttccccggctggaagggctactttgcgcgttcaggagctggttgggcccatgctcgcaatgcactcgtggctgctgcaagggaggctcagagaatgggcgtgaagttcgtaactggcactcctcagggcagagtagtcactctaatatttgagaataacgatgtcaaaggtgccgttaccggagacggcaagatttggcgtgcagagcgcacattcctctgcgccggtgccagcgctggtcagttcctcgacttcaagaatcagttgcgtccaacggcatggacgctggttcatattgctctgaagcctgaggagcgggctctttacaagaatatcccagttatcttcaacattgagagggggttcttcttcgaaccagatgaggagcgcggtgagattaagatctgcgacgaacatccggggtataccaatatggtacagtctgccgacggcacgatgatgagcattccttttgaaaagactcagattcctaaagaagccgagacgagggttagagctctgcttaaagagacgatgccacagcttgcagaccgtccattcagtttcgccaggatttgctggtgcgccgacactgccaaccgggagttcttgatcgatcgccatcctcagtaccattcgcttgtgctgggctgcggcgcttccggcagaggattcaaatatctaccttcaattggcaatctcatcgttgatgctatggaaggcaaggtccctcaaaagatccacgaactgattaaatggaacccagatattgctgccaatcgcaactggagggatactttggggagattcgggggtcccaacagagtaatggacttccacgacgtcaaggagtggacaaatgtacaatatagagatatttccaagttataa

SEQ ID NO: 131 - protein, 437 aa, Aspergillus terreus
MPVTKSSSILIIGAGTWGCSTALHLARRGYTNVTVLDPYPVPSAISAGNDVNKIISSGQYSSKKDEVEVNEIIAEQAFNGWKNDPIFKPYYHDTGVVMSATTQEGLERLGVRVRPEDEPDVAELTRPEQFRQLAPGVLKGNFPGWRGYHIRSNAGWAHARNALVAAAREAQRLGVRFVAGSPQGRVITLIFENNDVKGAVTADGKIWRAEQTILCAGAAAGQFLDFKDQLRPTAWTLVHIQLKPEERAQYKNMPVVFNIEKGFFFEPDEERGEIKICDEHPGYTNMTTGADGRVRSIPFEKTQVPREAEMRVRKLLSETMPQLADRPFSFARICWCADTPNREFIIDRHPEYPSLVLGCGASGRGFKYLPSIGSIIADAMEDKTPAKIHKLIRWSPEIAINRNWGDRLGRFGGPNRVMDFNEVKEWTNVTQRDISKL

SEQ ID NO: 132 - DNA, 1314 bp, Aspergillus terreus
atgccagtcaccaagtcttcgtcgatattgatcatcggggcgggcacctggggttgctcaactgccctgcatcttgcccgcagaggatacaccaatgtcactgtccttgacccgtacccggttccatcagccatttcggccggcaacgacgtcaacaagatcatctcgtccggccagtacagcagcaagaaggacgaggtcgaagtcaatgagattatcgccgaacaggccttcaatggctggaaaaatgaccccatcttcaagccgtactaccacgacaccggcgtcgtgatgtccgccaccacacaggaaggattggagcgtctgggggtccgcgtgcgacctgaagatgaacccgatgtagccgaattgactcggccggagcagttccgccagctggcccccggcgtcttgaagggtaacttccccggttggagggggtaccacattcgctcaaacgcgggctgggcgcatgcgcgcaacgccctggtcgccgcggcgcgggaggcacagcgcctgggtgtgcgcttcgtcgcgggatcgccgcagggcagagtcatcacgttgatttttgagaacaacgatgtgaagggtgccgtcacggcggacggcaagatctggcgggccgagcagactatcctctgcgctggtgcggccgccggccagtttctggatttcaaggaccaactgcgtcccactgcgtggactctggtccacatccagttgaagccggaagagcgtgcccagtataaaaacatgccggtggtcttcaacatcgagaaggggttcttcttcgagccggatgaggagcgtggtgaaatcaagatctgcgacgaacaccccgggtacacgaatatgaccacgggggccgacggccgcgtgaggagcattcccttcgagaagacgcaggttcctcgagaagcggagatgcgcgtccgcaagcttctgtctgaaacgatgcctcagcttgcggaccggccgttcagtttcgcaaggatctgctggtgtgcggatacccccaatcgcgagtttatcattgaccgtcatcccgaatacccgtcgcttgttcttgggtgtggtgcttcaggacgaggcttcaaatatcttccctcgatcggaagcatcatcgcagacgccatggaggacaaaaccccggcaaaaatccacaagctgatccgctggagcccggaaatcgcgatcaaccgtaactggggggacagattaggtcgatttggagggcccaaccgggtcatggatttcaatgaagtgaaggagtggactaatgtcacccaaagggacatctcgaagttatag

SEQ ID NO: 133 - protein, 437 aa, Coniochaeta sp.
MTSNRADTRVIVVGGGGTIGSSTALHLVRSGYAPANITVLDTFEIPSAQSAGHDLNKIMGIDLRNKVDLQMSLEARQMWKEDELFQPFFHNTGRMDCEHTPEGIEKLKKLYQKLHDAGAGLEKTHAWLDNEDEILSKMPLLQRDQIQGWKAIWSQDGGWLAAAKAINAIGQFLKERGVKFGFGGAGSFKQPLFDDEGTTCIGVETADGTKYYADKVVLAAGAWSPTLVDLEDQCCSKAWVYAHIQLTPEEAAEYKGVPVVYNGEFGFFFEPDEFGVIKVCDEFPGFSRFKEHQPYGAPSPKRISVPRSHAKHPTDTYPDASEVSIKKAIATFLPRFQDKELFNRALCWCTDTADAALLMCEHPKWKNFILATGDSGHSFKILPNVGKYVVELIEGRLPEEMAYQWRWRPGGDALKSRRAAPPKDLADMPGWKHDPKL

SEQ ID NO: 134 - DNA, 1314 bp, Coniochaeta sp.
atgacgtcgaatcgtgcagatacaagggtgattgtcgtcggtggcggaggaacgattggttcctcgacagcgctgcatcttgtgaggagtggttatgctcccgcaaatatcacggtcttggacacatttgagattccatcggctcaatcagccggccatgatctcaacaagatcatgggaatagatctgcgcaacaaggtggacctgcaaatgagtctagaggctagacagatgtggaaggaggatgagttattccagcccttctttcacaataccggcagaatggactgcgaacacacgcctgagggtatcgagaaactgaaaaagctgtaccagaaactgcacgatgccggtgcgggtctggagaagactcatgcctggttggacaacgaggatgagatcttatccaagatgccgttgcttcaacgtgaccaaatacaaggatggaaagcaatatggagtcaagatggcggctggttagctgcggcaaaggccatcaatgcgatcggacagttcttgaaagaacgtggtgtaaagttcggattcggcggcgctggatccttcaagcaaccccttttcgacgatgaaggcacaacttgcattggcgttgagacggcagatggtaccaaatattacgctgacaaggtggtcttagcagctggcgcatggagcccaaccctggtggacctggaagatcaatgttgctcgaaggcttgggtgtatgctcatattcagttgacgcctgaagaggccgctgagtataagggtgtcccagttgtgtataatggcgaatttggcttcttctttgagcctgatgagtttggtgtaataaaggtgtgcgacgagttcccaggattctcgcgcttcaaggaacatcaaccctatggcgccccatctccgaaacggatatcagtaccacgatcgcacgccaagcatcccacagacacttatccagacgcatccgaagtcagcatcaaaaaagcaatcgcgacgtttctccctcgatttcaggacaaggagctcttcaatcgcgccttgtgctggtgtacagacactgcggacgctgctctcttgatgtgtgaacaccccaaatggaagaatttcattctagcgaccggcgacagcggacactcattcaaaatcttgcctaacgtcggaaaatacgtagtcgagttgatagagggccgcctgccggaggaaatggcttatcaatggaggtggcggccaggaggcgatgcactcaagtctagacgtgcggcaccgccaaaagatcttgcagacatgccaggatggaaacatgatccgaaattgtaa

SEQ ID NO: 135 - protein, 437 aa, Phaeosphaeria nodorum
MAPSRANTSVIVVGGGGTIGSSTALHLVRSGYTPSNVTVLDAYPIPSSQSAGNDLNKIMGVDLRNPVDLQLALEARQMWNEDELFKKFFHNTGRLDCAHGEKDIAKLKSLYQKLVDAGLDATNEWLDSEDEILKRMPLLSRDQIKGWKAIFSKDGGWLAAAKAINAVGEYLRDQGVRFGFYGAGSFKAPLLAEGVCIGVETVDGTRYYADKVVLAAGAWSPTLVELHEQCVSKAWVYGHIQLTPEEAARYKNSPVVYNGDVGFFFEPNEHGVIKVCDEFPGFTRFKMHQPFGAKAPKRISVPRSHAKHPTDTIPDASDVSIRRAIATFMPQFKNKKMFNQAMCWCTDTADAALLICEHPEWKNFVLATGDSGHSFKLLPNIGKHVVELLEGTLADDLAHAWRWRPGSGDALKSRRSAPAKDLADMPGWNHDKPRANL

SEQ ID NO: 136 - DNA, 1314 bp, Phaeosphaeria nodorum
atggccccgtcgcgtgctaatacgtcggtcattgtggttggtggtggtggtacgattggctcatctacggctctgcatctggtccgctcaggctataccccgtcgaacgtgacggttctggatgcatacccgattccgagctctcagagcgctggcaacgacctgaataaaatcatgggtgtcgatctgcgtaatccggtggatctgcagctggctctggaagcgcgccaaatgtggaacgaagacgaactgttcaagaagtttttccataacaccggccgtctggattgcgcgcacggtgaaaaagatattgccaaactgaagagcctgtatcagaaactggtggatgcgggtctggacgccacgaacgaatggctggatagtgaagacgaaatcctgaaacgtatgccgctgctgtcccgcgatcaaattaaaggctggaaggcgatcttttcaaaagacggtggttggctggcagcagcaaaggcaattaatgcagttggtgaatatctgcgtgatcagggcgtccgcttcggtttttacggcgccggttctttcaaagcaccgctgctggctgaaggcgtctgcatcggtgtcgaaaccgtggatggcacgcgctattacgcagacaaagtggttctggctgcaggtgcatggtcgccgaccctggttgaactgcatgaacagtgtgtgagcaaagcgtgggtttacggccacattcaactgacgccggaagaagccgcacgttataagaacagcccggtcgtgtacaatggcgatgtgggctttttctttgaaccgaacgaacatggcgttatcaaagtctgcgatgaatttccgggttttacccgcttcaagatgcaccagccgtttggtgccaaagcaccgaagcgtattagtgtgccgcgctcccatgccaaacacccgaccgatacgatcccggatgcaagtgacgtttccattcgtcgcgctatcgcgacctttatgccgcagttcaagaacaaaaagatgttcaaccaagcgatgtgctggtgtaccgatacggccgacgctgcgctgctgatttgtgaacatccggaatggaaaaactttgttctggcgaccggcgattcaggtcattcgttcaaactgctgccgaatatcggcaagcacgttgtcgaactgctggagggtacgctggcagatgacctggcacacgcatggcgttggcgtccgggtagtggtgatgcactgaaaagccgtcgctctgctccggcgaaagacctggctgatatgccgggctggaaccatgacaaaccgcgtgctaatctgtaa

SEQ ID NO: 137 - protein, 441 aa, Neocosmospora vasinfecta
MTTPRKETTVLIIGGGGTIGSSTALHLLRAGYTPSNITVLDTYPIPSAQSAGNDLNKIMGIDLRNKVDLQLSLEARDMWRNDALFRPFFHNTGRLDCESSAEGVEKLRRLYQKLVEAGVGLEETHEWLDSEEAILEKAPLLQREEIEGWKAIWSEEGGWLAAAKAINAIGEELQRQGVRFGFGGAGSFKRPLFADDGTTCIGVETVDGTQYHADKVVLAAGAWSPALVDLEEQCCSKAWVYAHMQLTPEEAAVYKGCPVVYHGDVGFFFEPNENGVIKVCDEFPGFTRFKQHQPYGAPAPKPVSVPRSHAKHPTDTYPDASEESIKRAVSTFLPRFKDKPLFNRALCWCTDTADSALLICEHPRWKNFILATGDSGHSFKLLPIIGKHVVELVEGRLADDLAEAWRWRPGQGDARKSIRAAPAKDLADMPGWKHDQDSESR

SEQ ID NO: 138 - DNA, 1326 bp, Neocosmospora vasinfecta
atgacgaccccgcgtaaagaaacgacggtcctgattattggtggtggtggcacgattggtagctcgacggctctgcatctgctgcgtgccggctataccccgtctaacattaccgtgctggatacgtacccgatcccgagtgcccagtccgcaggcaacgacctgaataaaattatgggtatcgatctgcgcaataaagttgatctgcaactgagcctggaagcccgtgatatgtggcgcaacgacgcactgtttcgtccgtttttccataataccggccgcctggactgcgaaagctctgctgaaggcgtggaaaaactgcgtcgcctgtatcagaaactggtggaagcaggcgttggtctggaagaaacgcacgaatggctggatagcgaagaagctattctggaaaaagcgccgctgctgcaacgtgaagaaattgaaggttggaaagccatctggtctgaagaaggcggttggctggcggccgcaaaagctattaacgcgatcggcgaagaactgcagcgtcaaggcgttcgcttcggttttggcggtgccggtagttttaaacgcccgctgttcgcagatgacggcaccacgtgtatcggtgtcgaaaccgtggatggcacgcagtatcatgcggacaaagtggttctggctgcaggtgcttggtcaccggcgctggtcgatctggaagaacagtgctgttcgaaagcctgggtgtacgcacacatgcaactgaccccggaagaagccgcagtttataaaggctgcccggtcgtgtaccacggcgatgtcggctttttctttgaaccgaacgaaaatggcgttattaaagtctgtgacgaattcccgggttttacgcgtttcaaacagcatcaaccgtatggtgccccggcaccgaaacctgtgagtgttccgcgctcccatgcgaaacacccgaccgatacgtacccggacgcttcagaagaatcgatcaaacgtgccgtgagtacctttctgccgcgcttcaaagataaaccgctgtttaaccgtgcactgtgctggtgtaccgatacggccgactccgcactgctgatttgcgaacacccgcgctggaaaaattttatcctggcgaccggcgatagcggtcattctttcaaactgctgccgattatcggcaaacacgttgtcgaactggttgaaggtcgtctggcggatgacctggctgaagcgtggcgttggcgtccgggtcagggtgatgcacgtaaaagcattcgcgctgcgccggcgaaagacctggcggatatgccgggctggaaacacgaccaagactcggaatcacgctga

SEQ ID NO: 139 - protein, 438 aa, Aspergillus nidulans
MTPRANTKIIVVGGGGTMGSSTALHLLRAGYTPSNITVLDTCPIPSAQSAGYDLNKIMGIDLRNKPDLQLSLEALDMWKNDPLFKPFFHNVGMIDVSSTEEGIEKLRKLYQSLLDAGIGLEKTNFMLESEDEILAKAPHFTQEQIKGWKGLFCGDGGWLAAAKAINAIGQFLKEQGVKFGFGGAGTFKKPLFADAHEKTCIGVETVDGTKYYADKVVLAAGAWSSTLVDLEEQCVSKAWVFAHIQLTPAEAAAYKNTPVIYDGDYGFFFEPNENGIIKVCDEFPGFTHFKMHQPYGSPAPKPISVPRSHAKHPTDTYPHASEVTIKKAINRFLPRFNDKELFNRAMCWCTDTADANLLVCEHPRWKGFYLATGDSGHSFKLLPNIGKHVVELLEERLESVFKDAWRWRPGSGDALKSRRAAPAKDLADMPGWRNEAKM

SEQ ID NO: 140 - DNA, 1317 bp, Aspergillus nidulans
atgacgccccgagccaacaccaaaatcattgtcgtcggcggcggcggcacaatgggctcgtcgacagccctacacctcctgcgcgccggctacacgccgtccaacattacagtgctcgacacgtgccctatcccctccgcacagtctgcaggctacgacctgaacaaaatcatgggcatcgatctgcgcaacaagcctgatttacagctctctcttgaggcgctggacatgtggaaaaatgatcctctcttcaagccgtttttccacaatgttggaatgatcgacgtctcttcaacagaggaaggcatcgagaaacttcggaagctgtaccagtctcttctcgacgcaggcattgggctcgagaagacgaatttcatgctggaaagtgaagacgagatcctggctaaagcgccgcatttcacgcaggagcagattaaaggctggaaaggcctgttctgtggcgacggcggctggctcgctgcagccaaagccatcaatgccattgggcagttcctcaaggaacagggcgtcaagtttggattcggcggcgccggcacgttcaaaaagccactcttcgccgatgcccacgagaagacgtgcatcggcgtcgagactgtagacggcacaaagtactacgccgacaaggtcgttctagcagctggtgcctggagttcgacgttggtcgatctggaggagcagtgcgtttcaaaggcctgggtctttgcccacatccaactgacgcccgctgaagcagccgcgtataagaacactcctgttatatacgacggtgactatgggtttttctttgagccgaatgaaaacggcatcataaaagtctgtgacgaattccctggcttcacgcatttcaaaatgcaccagccgtacggctcgccggcgcccaaacccatctctgtgcctcgttcccatgcgaagcaccccacagatacatacccgcacgcgtcggaggtcacgatcaaaaaggctatcaaccggttcctgccgaggttcaatgacaaggaactgtttaacagggccatgtgctggtgcaccgataccgcggatgcaaatctgcttgtttgtgagcatccacgctggaaggggttttatcttgcaacaggggacagtgggcattcgttcaagttgctgccgaatattggaaagcatgttgtcgagttattggaggagaggctggaaagtgtgtttaaggatgcttggaggtggaggcctggcagtggggatgcattaaaaagtagacgggctgcgcctgcgaaggacctggcggatatgccggggtggaggaatgaggcaaagatgtag

SEQ ID NO: 141 - protein, 437 aa, Coniochaeta sp.
MTSNRADTRVIVVGGGGTIGSSTALHLVRSGYAPANITVLDTFEIPSAQSAGHDLNKIMGIDHRNKVDLQMSLEARQMWKEDELFQPFFHNTGRMDCEHTPKGIEKLKKLYQKLHDAGAGLEKTHAWLDNEDEILSKMPLLQRDQIQGWKAIWSQDGGWLAAAKAINAIGQFLKERGVKFGFGGAGSFKQPLFDDEGTTCIGVETADGTKYYADKVVLAAGAWSPTLVDLEDQCCSKAWVYAHIQLTPEEAAEYKGVPVVYNGEFGFFFEPDEFGVIKVCDEFPGFSRFKEHQPYGAPSPKRISVPRSHAKHPTDTYPDASEVSIKKAIATFLPRFQDKELFNRALCWCTDTADSALLMCEHPKWKNFILATGDSGHSFKILPNVGKYVVELIEGRLPEEMAYQWRWRPGGDALKSRRAAPPKDLADMPGWKHDPKL

SEQ ID NO: 142 - DNA, 1314 bp, Coniochaeta sp.
atgacgtcgaatcgtgcagatacaagggtgattgtcgtcggtggcggaggaacgattggttcctcgacagcgctgcatcttgtgaggagtggttatgctcccgcaaatatcacggtcttggacacatttgagattccatcggctcaatcagccggccatgatctcaacaagatcatgggaatagatcatcgcaacaaggtggacctgcaaatgagtctagaggctagacagatgtggaaggaggatgagttattccagcccttctttcacaataccggcagaatggactgcgaacacacgcctaagggtatcgagaaactgaaaaagctgtaccagaaactgcacgatgccggtgcgggtctggagaagactcatgcctggttggacaacgaggatgagatcttatccaagatgccgttgcttcaacgtgaccaaatacaaggatggaaagcaatatggagtcaagatggcggctggttagctgcggcaaaggccatcaatgcgatcggacagttcttgaaagaacgtggtgtaaagttcggattcggcggcgctggatccttcaagcaaccccttttcgacgatgaaggcacaacttgcattggcgttgagacggcagatggtaccaaatattacgctgacaaggtggtcttagcagctggcgcatggagcccaaccctggtggacctggaagatcaatgttgctcgaaggcttgggtgtatgctcatattcagttgacgcctgaagaggccgctgagtataagggtgtcccagttgtgtataatggcgaatttggcttcttctttgagcctgatgagtttggtgtaataaaggtgtgcgacgagttcccaggattctcgcgcttcaaggaacatcaaccctatggcgccccatctccgaaacggatatcagtaccacgatcgcacgccaagcatcccacagacacttatccagacgcatccgaagtcagcatcaaaaaagcaatcgcgacgtttctccctcgatttcaggacaaggagctcttcaatcgcgccttgtgctggtgtacagacactgcggactctgctctcttgatgtgtgaacaccccaaatggaagaatttcattctagcgaccggcgacagcggacactcattcaaaatcttgcctaacgtcggaaaatacgtagtcgagttgatagagggccgcctgccggaggaaatggcttatcaatggaggtggcggccaggaggcgatgcactcaagtctagacgtgcggcaccgccaaaagatcttgcagacatgccaggatggaaacatgatccgaaattgtaa

SEQ ID NO: 143 - protein, 437 aa, Eupenicillium terrenum
MAHSRASTKVVVVGGGGTIGSSTALHLIRSGYTPSNITVLDVYKTPSLQSAGHDLNKIMGIDHRNGPDLQLSLESLDMWQNDELFKPFFHQVGMIDCSSSKEGIEKLRRLYQKLLDAGIGLEKTNVWLESEDEILAKAPNFTREQVKGWKGLFCTDGGWLAAAKAINAIGIFLQDKGVKFGFGDAGTFQQPLFAADGKTCIGLETTDGTKYFADKVVLAAGAWSPTLVDLEDQCVSKAWVFAHIQLTPKEADAYKNVPVVYDGEYGFFFEPDEYGVIKVCDEFPGFSRFKLHQPYGAASPKMISVPRSHAKHPTDTYPDASEVTIRKAIARFLPEFKDKELFNRTMCWCTDTADSNLLICEHPKWKNFILATGDSGHSFKLLPNIGKYVVELLEGSLSQEMAGAWRWRPGGDALRSRRGAPAKDLAEMPGWKHDAHL

SEQ ID NO: 144 - DNA, 1314 bp, Eupenicillium terrenum
atggctcattcgcgtgcaagcaccaaagtcgtcgtggttgggggaggtggtacgatcgggtcttcgacggctctgcacttaatccgctctggatataccccctcaaatatcaccgtgcttgacgtatacaagaccccttcattgcaatctgcaggacatgatttgaacaagatcatgggcattgatcatcgcaacgggcctgacttgcagctttcgctggaatcactcgacatgtggcaaaacgatgagttgttcaagccattctttcaccaagtgggcatgattgattgttcgtcatccaaagagggtattgaaaaacttcgacgattataccagaaactcctcgatgcgggcattgggctggagaagacgaacgtttggctggaatctgaagatgagatcctcgccaaagcgccgaatttcacgcgtgaacaagtcaaggggtggaaaggcttattttgcactgatggaggctggcttgctgcagccaaggctatcaatgcgatcggaattttcctccaggacaaaggtgtcaagtttggctttggagatgctggtacctttcagcaacctctgttcgccgctgatggaaaaacttgcatcggacttgaaactacagacggaaccaagtactttgctgacaaggttgtcttggctgctggtgcgtggagtcccaccttggtggatctagaagatcagtgtgtttcaaaggcctgggttttcgctcatattcaactcacacccaaagaagcggacgcgtacaagaatgtgcctgtggtctatgatggtgaatatgggttctttttcgaacccgacgagtatggggtgatcaaagtctgtgacgagttccctggtttctctcgcttcaaactgcatcaaccgtacggggctgcatctcccaagatgatatccgtaccgcgatcacacgccaagcatcccacagatacctaccctgatgcctccgaagtcaccatacgcaaagcgatcgcaaggttcctgccagaatttaaagacaaggagctcttcaaccgtaccatgtgctggtgtacagatacggccgattctaacttattgatttgcgaacacccgaagtggaagaatttcattctggccactggagatagcggacattccttcaagctgttgccaaacatcgggaaatacgtagttgagcttttagagggatctctatcgcaggaaatggctggtgcctggagatggagacccggaggtgatgctcttagatctagacgcggtgctccggcaaaggatcttgctgagatgccgggatggaagcatgatgcacatttgtga

SEQ ID NO: 145 - protein, 437 aa, Eupenicillium terrenum
MAHSRASTKVVVVGGGGTIGSSTALHLIRSGYTPSNITVLDVYKTPSLQSAGHDLNKIMGIRLRNGPDLQLSLESLDMWQNDELFKPFFHQVGMIDCSSSKEGIENLRRKYQTLLDAGIGLEKTNVWLESEDEILAKAPNFTREQVKGWKGLFCTDGGWLAAAKAINAIGIFLQDKGVKFGFGGAGTFQQPLFAADGKTCIGLETTDGTKYFADKVVLAAGAWSPTLVDLEDQCVSKAWVFAHIQLTPKEADAYKNVPVVYDGEYGFFFEPNEYGVIKVCDEFPGFSRFKLHQPYGAASPKMISVPRSHAKHPTDTYPDASEVTIRKAIARFLPEFKDKELFNRTMCWCTDTADANLLICEHPKWKNFILATGDSGHSFKLLPNIGKHVVELLEGSLSQEMAGAWRWRPGGDALRSRRGAPAKDLAEMPGWKHDAHL

SEQ ID NO: 146 - DNA, 1314 bp, Eupenicillium terrenum
atggctcattcgcgtgcaagcaccaaagtcgtcgtggttgggggaggtggtacgatcgggtcttcgacggctctgcacttaatccgctctggatataccccctcaaatatcaccgtgcttgacgtatacaagaccccttcattgcaatctgcaggacatgatttgaacaagatcatgggcattcgattgcgcaacgggcctgacttgcagctttcgctggaatcactcgacatgtggcaaaacgatgagttgttcaagccattctttcaccaagtgggcatgattgattgttcgtcatccaaagagggtattgaaaatcttcgacgaaaataccagaccctcctcgatgcgggcattgggctggagaagacgaacgtttggctggaatctgaagatgagatcctcgccaaagcgccgaatttcacgcgtgaacaagtcaaggggtggaaaggcttattttgcactgatggaggctggcttgctgcagccaaggctatcaatgcgatcggaattttcctccaggacaaaggtgtcaagtttggctttggaggtgctggaacatttcagcaacctctgttcgccgctgatggaaaaacttgcatcggacttgaaactacagacggaaccaagtactttgctgacaaggttgtcttggctgctggtgcgtggagtcccaccttggtggatctagaagatcagtgtgtttcaaaggcctgggttttcgctcatattcaactcacacccaaagaagcggacgcgtacaagaatgtgcctgtggtctatgatggtgaatatgggttcttttttgagcccaacgagtatggggtgatcaaagtctgtgacgagttccctggtttctctcgcttcaaactgcatcaaccgtacggggctgcatctcccaagatgatatccgtaccgcgatcacacgccaagcatcccacagatacctaccctgatgcctccgaagtcaccatacgcaaagcgatcgcaaggttcctgccagaatttaaagacaaggagctcttcaaccgtaccatgtgctggtgtacagatacggccgatgctaacttattgatttgcgaacacccgaagtggaagaatttcattctggccactggagatagcggacattccttcaagctgttgccaaacatcgggaaacacgttgttgagcttttagagggatctctatcgcaggaaatggctggtgcctggagatggagacccggaggtgatgctcttagatctagacgcggtgctccggcaaaggatcttgctgagatgccgggatggaagcatgatgcacatttgtga

SEQ ID NO: 147 - protein, 438 aa, Aspergillus nidulans
MTPRANTKIIVVGGGGTMGSSTALHLLRAGYTPSNITVLDTCPIPSAQSAGYDLNKIMSIRLRNKPDLQLSLEALDMWKNDPLFKPFFHNVGMIDVSSTEEGIEGLRKKYQSLLDAGIGLEKTNFMLESEDEILAKAPHFTQEQIKGWKGLFCGDGGWLAAAKAINAIGQFLKEQGVKFGFGGAGTFKKPLFADAHEKTCIGVETVDGTKYYADKVVLAAGAWSSTLVDLEEQCVSKAWVFAHIQLTPAEAAAYKNTPVIYDGDYGFFFEPNENGIIKVCDEFPGFTHFKMHQPYGSPAPKPISVPRSHAKHPTDTYPHASEVTIKKAINRFLPRFNDKELFNRAMCWCTDTADANLLVCEHPRWKGFYLATGDSGHSFKLLPNIGKHVVELLEERLESVFKDAWRWRPGSGDALKSRRAAPAKDLADMPGWRNEAKM

SEQ ID NO: 148 - DNA, 1317 bp, Aspergillus nidulans
atgacgccccgagccaacaccaaaatcattgtcgtcggcggcggcggcacaatgggctcgtcgacagccctacacctcctgcgcgccggctacacgccgtccaacattacagtgctcgacacgtgccctatcccctccgcacagtctgcaggctacgacctgaacaaaatcatgagcatcaggctgcgcaacaagcctgatttacagctctctcttgaggcgctggacatgtggaaaaatgatcctctcttcaagccgtttttccacaatgttggaatgatcgacgtctcttcaacagaggaaggcatcgagggtcttcggaagaaataccagtctcttctcgacgcaggcattgggctcgagaagacgaatttcatgctggaaagtgaagacgagatcctggctaaagcgccgcatttcacgcaggagcagattaaaggctggaaaggcctgttctgtggcgacggcggctggctcgctgcagccaaagccatcaatgccattgggcagttcctcaaggaacagggcgtcaagtttggattcggcggcgccggcacgttcaaaaagccactcttcgccgatgcccacgagaagacgtgcatcggcgtcgagactgtagacggcacaaagtactacgccgacaaggtcgttctagcagctggtgcctggagttcgacgttggtcgatctggaggagcagtgcgtttcaaaggcctgggtctttgcccacatccaactgacgcccgctgaagcagccgcgtataagaacactcctgttatatacgacggtgactatgggtttttctttgagccgaatgaaaacggcatcataaaagtctgtgacgaattccctggcttcacgcatttcaaaatgcaccagccgtacggctcgccggcgcccaaacccatctctgtgcctcgttcccatgcgaagcaccccacagatacatacccgcacgcgtcggaggtcacgatcaaaaaggctatcaaccggttcctgccgaggttcaatgacaaggaactgtttaacagggccatgtgctggtgcaccgataccgcggatgcaaatctgcttgtttgtgagcatccacgctggaaggggttttatcttgcaacaggggacagtgggcattcgttcaagttgctgccgaatattggaaagcatgttgtcgagttattggaggagaggctggaaagtgtgtttaaggatgcttggaggtggaggcctggcagtggggatgcattaaaaagtagacgggctgcgcctgcgaaggacctggcggatatgccggggtggaggaatgaggcaaagatgtag

SEQ ID NO: 149 - protein, 477 aa, Cryptococcus neoformans
MPPSRASTKVIVIGGGGTLGSSTALHLLRAGYTPSNITVLDTYLIPSAQSAGNDLNKIMGIRIRNPVDKQLSLEARDMWRNDEVFKPYFHNTGRLDCAHTPESIASLRKSYEAILKAGSGLEKTHHWLSTEDEILARAPLLDRKQIKGWKAIYSEDGGWLAAAKAINSIGQVLKEKGVTFGFGSAGSFKKPLFDEDGTKAIGIETVDGTQYFADKVVLAAGAWSPTLVDLEGQCCSKAWVYAHMQLTPEEAAEYKECPVVYNSELGFFFEPNEKGVIKVCDEFPGFTRFKQHQPYGASSTKHISFPRSHAKHPTDTIPDESDASIRRAISAFLPRFKEKELFNRALCWCTDTADANLLICEHPKWKNFILATGDSGHSFKILPNIGKHVVELIEGTLAEDLAESWRWRPGSGDPLISRRAAPARDLADLPGWNHDEPSDDDMDVKDVAVSLASVKIGENIGEKVVEDGARVGVKVLA

SEQ ID NO: 150 - DNA, 1434 bp, Cryptococcus neoformans
atgccaccttcgcgcgccagtactaaggtcatagttatcgggggcggtggtactctcgggtcctctactgctcttcaccttttacgagccggttacactccatccaacatcactgtgcttgacacgtatctaatcccatcagcacagtcggctggcaatgacctcaataagatcatgggtattcgtatcaggaatcctgtagataaacagttgagcctggaagcaagagacatgtggaggaatgatgaagttttcaagccttatttccacaacacgggaagacttgattgtgctcatacaccggagagcattgcatctttgcgtaaatcgtacgaggctatcttaaaggccgggagcgggctcgagaagacccaccattggctgagtacagaagatgaaatactggctagagcccctttgttggatcggaaacagatcaaaggatggaaagctatttacagcgaagatgggggctggcttgcggcggcgaaagctatcaacagtatcggccaggtgttgaaagagaaaggtgtgacattcggattcgggagtgcgggctcattcaagaaacccttgtttgacgaagacggtaccaaggccatcggcattgagacagttgatggtacgcaatattttgccgacaaggtcgttctggctgccggagcttggagtcctaccctcgtggatttggaagggcaatgctgttcaaaggcttgggtttacgcccatatgcaattgacaccagaagaggctgccgaatacaaggagtgtcctgtggtgtacaactctgaacttgggttcttcttcgagcccaatgaaaaaggagtcatcaaagtgtgcgacgaattcccagggttcacccgtttcaagcaacatcaaccttacggcgcctcctctactaaacacatctctttcccgcgctcccatgccaaacaccctaccgataccattccggacgagtcggacgcatctatccgccgtgctatctctgcctttttaccgagattcaaagaaaaagaactgttcaacagagcactgtgctggtgtacagataccgccgatgccaatcttttgatatgcgaacatcccaaatggaaaaattttatcttagctacaggggatagtggacattcattcaaaattcttcccaatatcggtaaacatgtcgttgaacttatagaaggtacccttgccgaggacttggctgagagctggagatggagacctggaagcggtgaccccctgatctctcgtcgggcagcccctgcaagggatcttgctgatcttccaggatggaaccatgatgagccctcggatgacgatatggatgtaaaggatgtcgctgtatcgcttgcttctgtgaaaattggcgaaaacatcggggagaaggttgtggaagatggagcacgagtcggagtcaaagttctagcttag

SEQ ID NO: 151 - protein, 437 aa, Coniochaeta sp.
MTSNRADTRVIVVGGGGTIGSSTALHLVRSGYAPANITVLDTFEIPSAQSAGHDLNKIMGIALRNKVDLQMSLEARQMWKEDELFQPFFHNTGRMDCEHTPEGIEDLKKQYQALHDAGAGLEKTHAWLDNEDEILSKMPLLQRDQIQGWKAIWSQDGGWLAAAKAINAIGQFLKERGVKFGFGGAGSFKQPLFDDEGTTCIGVETADGTKYYADKVVLAAGAWSPTLVDLEDQCCSKAWVYAHIQLTPEEAAEYKGVPVVYNGEFGFFFEPDEFGVIKVCDEFPGFSRFKEHQPYGAPSPKRISVPRSHAKHPTDTYPDASEVSIKKAIATFLPRFQDKELFNRALCWCTDTADAALLMCEHPKWKNFILATGDSGHSFKILPNVGKYVVELIEGRLPEEMAYQWRWRPGGDALKSRRAAPPKDLADMPGWKHDPKL

SEQ ID NO: 152 - DNA, 1314 bp, Coniochaeta sp.
atgacgtcgaatcgtgcagatacaagggtgattgtcgtcggtggcggaggaacgattggttcctcgacagcgctgcatcttgtgaggagtggttatgctcccgcaaatatcacggtcttggacacatttgagattccatcggctcaatcagccggccatgatctcaacaagatcatgggaatagcactgcgcaacaaggtggacctgcaaatgagtctagaggctagacagatgtggaaggaggatgagttattccagcccttctttcacaataccggcagaatggactgcgaacacacgcctgagggtatcgaggacctgaaaaagcagtaccaggcactgcacgatgccggtgcgggtctggagaagactcatgcctggttggacaacgaggatgagatcttatccaagatgccgttgcttcaacgtgaccaaatacaaggatggaaagcaatatggagtcaagatggcggctggttagctgcggcaaaggccatcaatgcgatcggacagttcttgaaagaacgtggtgtaaagttcggattcggcggcgctggatccttcaagcaaccccttttcgacgatgaaggcacaacttgcattggcgttgagacggcagatggtaccaaatattacgctgacaaggtggtcttagcagctggcgcatggagcccaaccctggtggacctggaagatcaatgttgctcgaaggcttgggtgtatgctcatattcagttgacgcctgaagaggccgctgagtataagggtgtcccagttgtgtataatggcgaatttggcttcttctttgagcctgatgagtttggtgtaataaaggtgtgcgacgagttcccaggattctcgcgcttcaaggaacatcaaccctatggcgccccatctccgaaacggatatcagtaccacgatcgcacgccaagcatcccacagacacttatccagacgcatccgaagtcagcatcaaaaaagcaatcgcgacgtttctccctcgatttcaggacaaggagctcttcaatcgcgccttgtgctggtgtacagacactgcggacgctgctctcttgatgtgtgaacaccccaaatggaagaatttcattctagcgaccggcgacagcggacactcattcaaaatcttgcctaacgtcggaaaatacgtagtcgagttgatagagggccgcctgccggaggaaatggcttatcaatggaggtggcggccaggaggcgatgcactcaagtctagacgtgcggcaccgccaaaagatcttgcagacatgccaggatggaaacatgatccgaaattgtaa

SEQ ID NO: 153 - protein, 437 aa, Coniochaeta sp.
MTSNRADTRVIVVGGGGTIGSSTALHLVRSGYAPANITVLDTFEIPSAQSAGHDLNKIMGIDLRNKVDLQMSLEARQMWKEDELFQPFFHNTGRMDCEHTPEGIEDLKKQYQALHDAGAGLEKTHAWLDNEDEILSKMPLLQRDQIQGWKAIWSQDGGWLAAAKAINAIGQFLKERGVKFGFGGAGSFKQPLFDDEGTTCIGVETADGTKYYADKVVLAAGAWSPTLVDLEDQCCSKAWVYAHIQLTPEEAAEYKGVPVVYNGEFGFFFEPDEFGVIKVCDEFPGFSRFKEHQPYGAPSPKRISVPRSHAKHPTDTYPDASEVSIKKAIATFLPRFQDKELFNRALCWCTDTADAALLMCEHPKWKNFILATGDSGHSFKILPNVGKYVVELIEGRLPEEMAYQWRWRPGGDALKSRRAAPPKDLADMPGWKHDPKL

SEQ ID NO: 154 - DNA, 1314 bp, Coniochaeta sp.
atgacgtcgaatcgtgcagatacaagggtgattgtcgtcggtggcggaggaacgattggttcctcgacagcgctgcatcttgtgaggagtggttatgctcccgcaaatatcacggtcttggacacatttgagattccatcggctcaatcagccggccatgatctcaacaagatcatgggaatagatctgcgcaacaaggtggacctgcaaatgagtctagaggctagacagatgtggaaggaggatgagttattccagcccttctttcacaataccggcagaatggactgcgaacacacgcctgagggtatcgaggacctgaaaaagcagtaccaggcactgcacgatgccggtgcgggtctggagaagactcatgcctggttggacaacgaggatgagatcttatccaagatgccgttgcttcaacgtgaccaaatacaaggatggaaagcaatatggagtcaagatggcggctggttagctgcggcaaaggccatcaatgcgatcggacagttcttgaaagaacgtggtgtaaagttcggattcggcggcgctggatccttcaagcaaccccttttcgacgatgaaggcacaacttgcattggcgttgagacggcagatggtaccaaatattacgctgacaaggtggtcttagcagctggcgcatggagcccaaccctggtggacctggaagatcaatgttgctcgaaggcttgggtgtatgctcatattcagttgacgcctgaagaggccgctgagtataagggtgtcccagttgtgtataatggcgaatttggcttcttctttgagcctgatgagtttggtgtaataaaggtgtgcgacgagttcccaggattctcgcgcttcaaggaacatcaaccctatggcgccccatctccgaaacggatatcagtaccacgatcgcacgccaagcatcccacagacacttatccagacgcatccgaagtcagcatcaaaaaagcaatcgcgacgtttctccctcgatttcaggacaaggagctcttcaatcgcgccttgtgctggtgtacagacactgcggacgctgctctcttgatgtgtgaacaccccaaatggaagaatttcattctagcgaccggcgacagcggacactcattcaaaatcttgcctaacgtcggaaaatacgtagtcgagttgatagagggccgcctgccggaggaaatggcttatcaatggaggtggcggccaggaggcgatgcactcaagtctagacgtgcggcaccgccaaaagatcttgcagacatgccaggatggaaacatgatccgaaattgtaa

SEQ ID NO: 155 - protein, 437 aa, Eupenicillium terrenum
MAHSRASTKVVVVGGGGTIGSSTALHLIRSGYTPSNITVLDVYKTPSLQSAGHDLNKIMGIDLRNGPDLQLSLESLDMWQNDELFKPFFHQVGMIDCSSSKEGIENLRRKYQTLLDAGIGLEKTNVWLESEDEILAKAPNFTREQVKGWKGLFCTDGGWLAAAKAINAIGIFLQDKGVKFGFGDAGTFQQPLFAADGKTCIGLETTDGTKYFADKVVLAAGAWSPTLVDLEDQCVSKAWVFAHIQLTPKEADAYKNVPVVYDGEYGFFFEPDEYGVIKVCDEFPGFSRFKLHQPYGAASPKMISVPRSHAKHPTDTYPDASEVTIRKAIARFLPEFKDKELFNRTMCWCTDTADANLLICEHPKWKNFILATGDSGHSFKLLPNIGKYVVELLEGSLSQEMAGAWRWRPGGDALRSRRGAPAKDLAEMPGWKHDAHL

SEQ ID NO: 156 - DNA, 1314 bp, Eupenicillium terrenum
atggctcattcgcgtgcaagcaccaaagtcgtcgtggttgggggaggtggtacgatcgggtcttcgacggctctgcacttaatccgctctggatataccccctcaaatatcaccgtgcttgacgtatacaagaccccttcattgcaatctgcaggacatgatttgaacaagatcatgggcattgatttgcgcaacgggcctgacttgcagctttcgctggaatcactcgacatgtggcaaaacgatgagttgttcaagccattctttcaccaagtgggcatgattgattgttcgtcatccaaagagggtattgaaaatcttcgacgaaaataccagaccctcctcgatgcgggcattgggctggagaagacgaacgtttggctggaatctgaagatgagatcctcgccaaagcgccgaatttcacgcgtgaacaagtcaaggggtggaaaggcttattttgcactgatggaggctggcttgctgcagccaaggctatcaatgcgatcggaattttcctccaggacaaaggtgtcaagtttggctttggagatgctggtacctttcagcaacctctgttcgccgctgatggaaaaacttgcatcggacttgaaactacagacggaaccaagtactttgctgacaaggttgtcttggctgctggtgcgtggagtcccaccttggtggatctagaagatcagtgtgtttcaaaggcctgggttttcgctcatattcaactcacacccaaagaagcggacgcgtacaagaatgtgcctgtggtctatgatggtgaatatgggttctttttcgaacccgacgagtatggggtgatcaaagtctgtgacgagttccctggtttctctcgcttcaaactgcatcaaccgtacggggctgcatctcccaagatgatatccgtaccgcgatcacacgccaagcatcccacagatacctaccctgatgcctccgaagtcaccatacgcaaagcgatcgcaaggttcctgccagaatttaaagacaaggagctcttcaaccgtaccatgtgctggtgtacagatacggccgatgctaacttattgatttgcgaacacccgaagtggaagaatttcattctggccactggagatagcggacattccttcaagctgttgccaaacatcgggaaatacgtagttgagcttttagagggatctctatcgcaggaaatggctggtgcctggagatggagacccggaggtgatgctcttagatctagacgcggtgctccggcaaaggatcttgctgagatgccgggatggaagcatgatgcacatttgtga

SEQ ID NO: 157 - protein, 437 aa, Coniochaeta sp.
MTSNRADTRVIVVGGGGTIGSSTALHLVRSGYAPANITVLDTFEIPSAQSAGHDLNKIMGIALRNKVDLQMSLEARQMWKEDELFQPFFHNTGRMDCEHTPEGIEDLKKLYQALHDAGAGLEKTHAWLDNEDEILSKMPLLQRDQIQGWKAIWSQDGGWLAAAKAINAIGQFLKERGVKFGFGGAGSFKQPLFDDEGTTCIGVETADGTKYYADKVVLAAGAWSPTLVDLEDQCCSKAWVYAHIQLTPEEAAEYKGVPVVYNGEFGFFFEPDEFGVIKVCDEFPGFSRFKEHQPYGAPSPKRISVPRSHAKHPTDTYPDASEVSIKKAIATFLPRFQDKELFNRALCWCTDTADAALLMCEHPKWKNFILATGDSGHSFKILPNVGKYVVELIEGRLPEEMAYQWRWRPGGDALKSRRAAPPKDLADMPGWKHDPKL

SEQ ID NO: 158 - DNA, 1314 bp, Coniochaeta sp.
atgacgtcgaatcgtgcagatacaagggtgattgtcgtcggtggcggaggaacgattggttcctcgacagcgctgcatcttgtgaggagtggttatgctcccgcaaatatcacggtcttggacacatttgagattccatcggctcaatcagccggccatgatctcaacaagatcatgggaatagcactgcgcaacaaggtggacctgcaaatgagtctagaggctagacagatgtggaaggaggatgagttattccagcccttctttcacaataccggcagaatggactgcgaacacacgcctgagggtatcgaggacctgaaaaagctgtaccaggcactgcacgatgccggtgcgggtctggagaagactcatgcctggttggacaacgaggatgagatcttatccaagatgccgttgcttcaacgtgaccaaatacaaggatggaaagcaatatggagtcaagatggcggctggttagctgcggcaaaggccatcaatgcgatcggacagttcttgaaagaacgtggtgtaaagttcggattcggcggcgctggatccttcaagcaaccccttttcgacgatgaaggcacaacttgcattggcgttgagacggcagatggtaccaaatattacgctgacaaggtggtcttagcagctggcgcatggagcccaaccctggtggacctggaagatcaatgttgctcgaaggcttgggtgtatgctcatattcagttgacgcctgaagaggccgctgagtataagggtgtcccagttgtgtataatggcgaatttggcttcttctttgagcctgatgagtttggtgtaataaaggtgtgcgacgagttcccaggattctcgcgcttcaaggaacatcaaccctatggcgccccatctccgaaacggatatcagtaccacgatcgcacgccaagcatcccacagacacttatccagacgcatccgaagtcagcatcaaaaaagcaatcgcgacgtttctccctcgatttcaggacaaggagctcttcaatcgcgccttgtgctggtgtacagacactgcggacgctgctctcttgatgtgtgaacaccccaaatggaagaatttcattctagcgaccggcgacagcggacactcattcaaaatcttgcctaacgtcggaaaatacgtagtcgagttgatagagggccgcctgccggaggaaatggcttatcaatggaggtggcggccaggaggcgatgcactcaagtctagacgtgcggcaccgccaaaagatcttgcagacatgccaggatggaaacatgatccgaaattgtaa

SEQ ID NO: 159 - protein, 437 aa, Coniochaeta sp.
MTSNRADTRVIVVGGGGTIGSSTALHLVRSGYAPANITVLDTFEIPSAQSAGHDLNKIMGIALRNKVDLQMSLEARQMWKEDELFQPFFHNTGRMDCEHTPEGIEDLKKYYQALHDAGAGLEKTHAWLDNEDEILSKMPLLQRDQIQGWKAIWSQDGGWLAAAKAINAIGQFLKERGVKFGFGGAGSFKQPLFDDEGTTCIGVETADGTKYYADKVVLAAGAWSPTLVDLEDQCCSKAWVYAHIQLTPEEAAEYKGVPVVYNGEFGFFFEPDEFGVIKVCDEFPGFSRFKEHQPYGAPSPKRISVPRSHAKHPTDTYPDASEVSIKKAIATFLPRFQDKELFNRALCWCTDTADAALLMCEHPKWKNFILATGDSGHSFKILPNVGKYVVELIEGRLPEEMAYQWRWRPGGDALKSRRAAPPKDLADMPGWKHDPKL

SEQ ID NO: 160 - DNA, 1314 bp, Coniochaeta sp.
atgacgtcgaatcgtgcagatacaagggtgattgtcgtcggtggcggaggaacgattggttcctcgacagcgctgcatcttgtgaggagtggttatgctcccgcaaatatcacggtcttggacacatttgagattccatcggctcaatcagccggccatgatctcaacaagatcatgggaatagcactgcgcaacaaggtggacctgcaaatgagtctagaggctagacagatgtggaaggaggatgagttattccagcccttctttcacaataccggcagaatggactgcgaacacacgcctgagggtatcgaggacctgaaaaagtattaccaggcactgcacgatgccggtgcgggtctggagaagactcatgcctggttggacaacgaggatgagatcttatccaagatgccgttgcttcaacgtgaccaaatacaaggatggaaagcaatatggagtcaagatggcggctggttagctgcggcaaaggccatcaatgcgatcggacagttcttgaaagaacgtggtgtaaagttcggattcggcggcgctggatccttcaagcaaccccttttcgacgatgaaggcacaacttgcattggcgttgagacggcagatggtaccaaatattacgctgacaaggtggtcttagcagctggcgcatggagcccaaccctggtggacctggaagatcaatgttgctcgaaggcttgggtgtatgctcatattcagttgacgcctgaagaggccgctgagtataagggtgtcccagttgtgtataatggcgaatttggcttcttctttgagcctgatgagtttggtgtaataaaggtgtgcgacgagttcccaggattctcgcgcttcaaggaacatcaaccctatggcgccccatctccgaaacggatatcagtaccacgatcgcacgccaagcatcccacagacacttatccagacgcatccgaagtcagcatcaaaaaagcaatcgcgacgtttctccctcgatttcaggacaaggagctcttcaatcgcgccttgtgctggtgtacagacactgcggacgctgctctcttgatgtgtgaacaccccaaatggaagaatttcattctagcgaccggcgacagcggacactcattcaaaatcttgcctaacgtcggaaaatacgtagtcgagttgatagagggccgcctgccggaggaaatggcttatcaatggaggtggcggccaggaggcgatgcactcaagtctagacgtgcggcaccgccaaaagatcttgcagacatgccaggatggaaacatgatccgaaattgtaa

SEQ ID NO: 161 - protein, 437 aa, Coniochaeta sp.
MTSNRADTRVIVVGGGGTIGSSTALHLVRSGYAPANITVLDTFEIPSAQSAGHDLNKIMGINLRNKVDLQMSLEARQMWKEDELFQPFFHNTGRMDCEHTPEGIEDLKKLYQALHDAGAGLEKTHAWLDNEDEILSKMPLLQRDQIQGWKAIWSQDGGWLAAAKAINAIGQFLKERGVKFGFGGAGSFKQPLFDDEGTTCIGVETADGTKYYADKVVLAAGAWSPTLVDLEDQCCSKAWVYAHIQLTPEEAAEYKGVPVVYNGEFGFFFEPDEFGVIKVCDEFPGFSRFKEHQPYGAPSPKRISVPRSHAKHPTDTYPDASEVSIKKAIATFLPRFQDKELFNRALCWCTDTADAALLMCEHPKWKNFILATGDSGHSFKILPNVGKYVVELIEGRLPEEMAYQWRWRPGGDALKSRRAAPPKDLADMPGWKHDPKL

SEQ ID NO: 162 - DNA, 1314 bp, Coniochaeta sp.
atgacgtcgaatcgtgcagatacaagggtgattgtcgtcggtggcggaggaacgattggttcctcgacagcgctgcatcttgtgaggagtggttatgctcccgcaaatatcacggtcttggacacatttgagattccatcggctcaatcagccggccatgatctcaacaagatcatgggaataaacctgcgcaacaaggtggacctgcaaatgagtctagaggctagacagatgtggaaggaggatgagttattccagcccttctttcacaataccggcagaatggactgcgaacacacgcctgagggtatcgaggacctgaaaaagctgtaccaggcactgcacgatgccggtgcgggtctggagaagactcatgcctggttggacaacgaggatgagatcttatccaagatgccgttgcttcaacgtgaccaaatacaaggatggaaagcaatatggagtcaagatggcggctggttagctgcggcaaaggccatcaatgcgatcggacagttcttgaaagaacgtggtgtaaagttcggattcggcggcgctggatccttcaagcaaccccttttcgacgatgaaggcacaacttgcattggcgttgagacggcagatggtaccaaatattacgctgacaaggtggtcttagcagctggcgcatggagcccaaccctggtggacctggaagatcaatgttgctcgaaggcttgggtgtatgctcatattcagttgacgcctgaagaggccgctgagtataagggtgtcccagttgtgtataatggcgaatttggcttcttctttgagcctgatgagtttggtgtaataaaggtgtgcgacgagttcccaggattctcgcgcttcaaggaacatcaaccctatggcgccccatctccgaaacggatatcagtaccacgatcgcacgccaagcatcccacagacacttatccagacgcatccgaagtcagcatcaaaaaagcaatcgcgacgtttctccctcgatttcaggacaaggagctcttcaatcgcgccttgtgctggtgtacagacactgcggacgctgctctcttgatgtgtgaacaccccaaatggaagaatttcattctagcgaccggcgacagcggacactcattcaaaatcttgcctaacgtcggaaaatacgtagtcgagttgatagagggccgcctgccggaggaaatggcttatcaatggaggtggcggccaggaggcgatgcactcaagtctagacgtgcggcaccgccaaaagatcttgcagacatgccaggatggaaacatgatccgaaattgtaa

SEQ ID NO: 163 - protein, 437 aa, Coniochaeta sp.
MTSNRADTRVIVVGGGGTIGSSTALHLVRSGYAPANITVLDTFEIPSAQSAGHDLNKIMGIDLRNKVDLQMSLEARQMWKEDELFQPFFHNTGRMDCEHTPEGIEDLKKLYQALHDAGAGLEKTHAWLDNEDEILSKMPLLQRDQIQGWKAIWSQDGGWLAAAKAINAIGQFLKERGVKFGFGGAGSFKQPLFDDEGTTCIGVETADGTKYYADKVVLAAGAWSPTLVDLEDQCCSKAWVYAHIQLTPEEAAEYKGVPVVYNGEFGFFFEPDEFGVIKVCDEFPGFSRFKEHQPYGAPSPKRISVPRSHAKHPTDTYPDASEVSIKKAIATFLPRFQDKELFNRALCWCTDTADAALLMCEHPKWKNFILATGDSGHSFKILPNVGKYVVELIEGRLPEEMAYQWRWRPGGDALKSRRAAPPKDLADMPGWKHDPKL

SEQ ID NO: 164 - DNA, 1314 bp, Coniochaeta sp.
atgacgtcgaatcgtgcagatacaagggtgattgtcgtcggtggcggaggaacgattggttcctcgacagcgctgcatcttgtgaggagtggttatgctcccgcaaatatcacggtcttggacacatttgagattccatcggctcaatcagccggccatgatctcaacaagatcatgggaatagatctgcgcaacaaggtggacctgcaaatgagtctagaggctagacagatgtggaaggaggatgagttattccagcccttctttcacaataccggcagaatggactgcgaacacacgcctgagggtatcgaggacctgaaaaagctgtaccaggcactgcacgatgccggtgcgggtctggagaagactcatgcctggttggacaacgaggatgagatcttatccaagatgccgttgcttcaacgtgaccaaatacaaggatggaaagcaatatggagtcaagatggcggctggttagctgcggcaaaggccatcaatgcgatcggacagttcttgaaagaacgtggtgtaaagttcggattcggcggcgctggatccttcaagcaaccccttttcgacgatgaaggcacaacttgcattggcgttgagacggcagatggtaccaaatattacgctgacaaggtggtcttagcagctggcgcatggagcccaaccctggtggacctggaagatcaatgttgctcgaaggcttgggtgtatgctcatattcagttgacgcctgaagaggccgctgagtataagggtgtcccagttgtgtataatggcgaatttggcttcttctttgagcctgatgagtttggtgtaataaaggtgtgcgacgagttcccaggattctcgcgcttcaaggaacatcaaccctatggcgccccatctccgaaacggatatcagtaccacgatcgcacgccaagcatcccacagacacttatccagacgcatccgaagtcagcatcaaaaaagcaatcgcgacgtttctccctcgatttcaggacaaggagctcttcaatcgcgccttgtgctggtgtacagacactgcggacgctgctctcttgatgtgtgaacaccccaaatggaagaatttcattctagcgaccggcgacagcggacactcattcaaaatcttgcctaacgtcggaaaatacgtagtcgagttgatagagggccgcctgccggaggaaatggcttatcaatggaggtggcggccaggaggcgatgcactcaagtctagacgtgcggcaccgccaaaagatcttgcagacatgccaggatggaaacatgatccgaaattgtaa

SEQ ID NO: 165 - protein, 437 aa, Coniochaeta sp.
MTSNRADTRVIVVGGGGTIGSSTALHLVRSGYAPANITVLDTFEIPSAQSAGHDLNKIMGIDLRNKVDLQMSLEARQMWKEDELFQPFFHNTGRMDCEHTPEGIEALKKLYQALHDAGAGLEKTHAWLDNEDEILSKMPLLQRDQIQGWKAIWSQDGGWLAAAKAINAIGQFLKERGVKFGFGGAGSFKQPLFDDEGTTCIGVETADGTKYYADKVVLAAGAWSPTLVDLEDQCCSKAWVYAHIQLTPEEAAEYKGVPVVYNGEFGFFFEPDEFGVIKVCDEFPGFSRFKEHQPYGAPSPKRISVPRSHAKHPTDTYPDASEVSIKKAIATFLPRFQDKELFNRALCWCTDTADAALLMCEHPKWKNFILATGDSGHSFKILPNVGKYVVELIEGRLPEEMAYQWRWRPGGDALKSRRAAPPKDLADMPGWKHDPKL

SEQ ID NO: 166 - DNA, 1314 bp, Coniochaeta sp.
atgacgtcgaatcgtgcagatacaagggtgattgtcgtcggtggcggaggaacgattggttcctcgacagcgctgcatcttgtgaggagtggttatgctcccgcaaatatcacggtcttggacacatttgagattccatcggctcaatcagccggccatgatctcaacaagatcatgggaatagatctgcgcaacaaggtggacctgcaaatgagtctagaggctagacagatgtggaaggaggatgagttattccagcccttctttcacaataccggcagaatggactgcgaacacacgcctgagggtatcgaggccctgaaaaagctgtaccaggcactgcacgatgccggtgcgggtctggagaagactcatgcctggttggacaacgaggatgagatcttatccaagatgccgttgcttcaacgtgaccaaatacaaggatggaaagcaatatggagtcaagatggcggctggttagctgcggcaaaggccatcaatgcgatcggacagttcttgaaagaacgtggtgtaaagttcggattcggcggcgctggatccttcaagcaaccccttttcgacgatgaaggcacaacttgcattggcgttgagacggcagatggtaccaaatattacgctgacaaggtggtcttagcagctggcgcatggagcccaaccctggtggacctggaagatcaatgttgctcgaaggcttgggtgtatgctcatattcagttgacgcctgaagaggccgctgagtataagggtgtcccagttgtgtataatggcgaatttggcttcttctttgagcctgatgagtttggtgtaataaaggtgtgcgacgagttcccaggattctcgcgcttcaaggaacatcaaccctatggcgccccatctccgaaacggatatcagtaccacgatcgcacgccaagcatcccacagacacttatccagacgcatccgaagtcagcatcaaaaaagcaatcgcgacgtttctccctcgatttcaggacaaggagctcttcaatcgcgccttgtgctggtgtacagacactgcggacgctgctctcttgatgtgtgaacaccccaaatggaagaatttcattctagcgaccggcgacagcggacactcattcaaaatcttgcctaacgtcggaaaatacgtagtcgagttgatagagggccgcctgccggaggaaatggcttatcaatggaggtggcggccaggaggcgatgcactcaagtctagacgtgcggcaccgccaaaagatcttgcagacatgccaggatggaaacatgatccgaaattgtaa

SEQ ID NO: 167 - protein, 437 aa, Coniochaeta sp.
MTSNRADTRVIVVGGGGTIGSSTALHLVRSGYAPANITVLDTFEIPSAQSAGHDLNKIMGIDLRNKVDLQMSLEARQMWKEDELFQPFFHNTGRMDCEHTPEGIEKLKKLYQALHDAGAGLEKTHAWLDNEDEILSKMPLLQRDQIQGWKAIWSQDGGWLAAAKAINAIGQFLKERGVKFGFGGAGSFKQPLFDDEGTTCIGVETADGTKYYADKVVLAAGAWSPTLVDLEDQCCSKAWVYAHIQLTPEEAAEYKGVPVVYNGEFGFFFEPDEFGVIKVCDEFPGFSRFKEHQPYGAPSPKRISVPRSHAKHPTDTYPDASEVSIKKAIATFLPRFQDKELFNRALCWCTDTADAALLMCEHPKWKNFILATGDSGHSFKILPNVGKYVVELIEGRLPEEMAYQWRWRPGGDALKSRRAAPPKDLADMPGWKHDPKL

SEQ ID NO: 168 - DNA, 1314 bp, Coniochaeta sp.
atgacgtcgaatcgtgcagatacaagggtgattgtcgtcggtggcggaggaacgattggttcctcgacagcgctgcatcttgtgaggagtggttatgctcccgcaaatatcacggtcttggacacatttgagattccatcggctcaatcagccggccatgatctcaacaagatcatgggaatagatctgcgcaacaaggtggacctgcaaatgagtctagaggctagacagatgtggaaggaggatgagttattccagcccttctttcacaataccggcagaatggactgcgaacacacgcctgagggtatcgagaaactgaaaaagctgtaccaggcactgcacgatgccggtgcgggtctggagaagactcatgcctggttggacaacgaggatgagatcttatccaagatgccgttgcttcaacgtgaccaaatacaaggatggaaagcaatatggagtcaagatggcggctggttagctgcggcaaaggccatcaatgcgatcggacagttcttgaaagaacgtggtgtaaagttcggattcggcggcgctggatccttcaagcaaccccttttcgacgatgaaggcacaacttgcattggcgttgagacggcagatggtaccaaatattacgctgacaaggtggtcttagcagctggcgcatggagcccaaccctggtggacctggaagatcaatgttgctcgaaggcttgggtgtatgctcatattcagttgacgcctgaagaggccgctgagtataagggtgtcccagttgtgtataatggcgaatttggcttcttctttgagcctgatgagtttggtgtaataaaggtgtgcgacgagttcccaggattctcgcgcttcaaggaacatcaaccctatggcgccccatctccgaaacggatatcagtaccacgatcgcacgccaagcatcccacagacacttatccagacgcatccgaagtcagcatcaaaaaagcaatcgcgacgtttctccctcgatttcaggacaaggagctcttcaatcgcgccttgtgctggtgtacagacactgcggacgctgctctcttgatgtgtgaacaccccaaatggaagaatttcattctagcgaccggcgacagcggacactcattcaaaatcttgcctaacgtcggaaaatacgtagtcgagttgatagagggccgcctgccggaggaaatggcttatcaatggaggtggcggccaggaggcgatgcactcaagtctagacgtgcggcaccgccaaaagatcttgcagacatgccaggatggaaacatgatccgaaattgtaa

SEQ ID NO: 169 - protein, 437 aa, Coniochaeta sp.
MTSNRADTRVIVVGGGGTIGSSTALHLVRSGYAPANITVLDTFEIPSAQSAGHDLNKIMGIDLRNKVDLQMSLEARQMWKEDELFQPFFHNTGRMDCEHTPEGIERLKKLYQALHDAGAGLEKTHAWLDNEDEILSKMPLLQRDQIQGWKAIWSQDGGWLAAAKAINAIGQFLKERGVKFGFGGAGSFKQPLFDDEGTTCIGVETADGTKYYADKVVLAAGAWSPTLVDLEDQCCSKAWVYAHIQLTPEEAAEYKGVPVVYNGEFGFFFEPDEFGVIKVCDEFPGFSRFKEHQPYGAPSPKRISVPRSHAKHPTDTYPDASEVSIKKAIATFLPRFQDKELFNRALCWCTDTADAALLMCEHPKWKNFILATGDSGHSFKILPNVGKYVVELIEGRLPEEMAYQWRWRPGGDALKSRRAAPPKDLADMPGWKHDPKL

SEQ ID NO: 170 - DNA, 1314 bp, Coniochaeta sp.
atgacgtcgaatcgtgcagatacaagggtgattgtcgtcggtggcggaggaacgattggttcctcgacagcgctgcatcttgtgaggagtggttatgctcccgcaaatatcacggtcttggacacatttgagattccatcggctcaatcagccggccatgatctcaacaagatcatgggaatagatctgcgcaacaaggtggacctgcaaatgagtctagaggctagacagatgtggaaggaggatgagttattccagcccttctttcacaataccggcagaatggactgcgaacacacgcctgagggtatcgagcgcctgaaaaagctgtaccaggcactgcacgatgccggtgcgggtctggagaagactcatgcctggttggacaacgaggatgagatcttatccaagatgccgttgcttcaacgtgaccaaatacaaggatggaaagcaatatggagtcaagatggcggctggttagctgcggcaaaggccatcaatgcgatcggacagttcttgaaagaacgtggtgtaaagttcggattcggcggcgctggatccttcaagcaaccccttttcgacgatgaaggcacaacttgcattggcgttgagacggcagatggtaccaaatattacgctgacaaggtggtcttagcagctggcgcatggagcccaaccctggtggacctggaagatcaatgttgctcgaaggcttgggtgtatgctcatattcagttgacgcctgaagaggccgctgagtataagggtgtcccagttgtgtataatggcgaatttggcttcttctttgagcctgatgagtttggtgtaataaaggtgtgcgacgagttcccaggattctcgcgcttcaaggaacatcaaccctatggcgccccatctccgaaacggatatcagtaccacgatcgcacgccaagcatcccacagacacttatccagacgcatccgaagtcagcatcaaaaaagcaatcgcgacgtttctccctcgatttcaggacaaggagctcttcaatcgcgccttgtgctggtgtacagacactgcggacgctgctctcttgatgtgtgaacaccccaaatggaagaatttcattctagcgaccggcgacagcggacactcattcaaaatcttgcctaacgtcggaaaatacgtagtcgagttgatagagggccgcctgccggaggaaatggcttatcaatggaggtggcggccaggaggcgatgcactcaagtctagacgtgcggcaccgccaaaagatcttgcagacatgccaggatggaaacatgatccgaaattgtaa

SEQ ID NO: 171 - protein, 437 aa, Coniochaeta sp.
MTSNRADTRVIVVGGGGTIGSSTALHLVRSGYAPANITVLDTFEIPSAQSAGHDLNKIMGIDLRNKVDLQMSLEARQMWKEDELFQPFFHNTGRMDCEHTPEGIEDLKKLYQKLHDAGAGLEKTHAWLDNEDEILSKMPLLQRDQIQGWKAIWSQDGGWLAAAKAINAIGQFLKERGVKFGFGGAGSFKQPLFDDEGTTCIGVETADGTKYYADKVVLAAGAWSPTLVDLEDQCCSKAWVYAHIQLTPEEAAEYKGVPVVYNGEFGFFFEPDEFGVIKVCDEFPGFSRFKEHQPYGAPSPKRISVPRSHAKHPTDTYPDASEVSIKKAIATFLPRFQDKELFNRALCWCTDTADAALLMCEHPKWKNFILATGDSGHSFKILPNVGKYVVELIEGRLPEEMAYQWRWRPGGDALKSRRAAPPKDLADMPGWKHDPKL

SEQ ID NO: 172 - DNA, 1314 bp, Coniochaeta sp.
atgacgtcgaatcgtgcagatacaagggtgattgtcgtcggtggcggaggaacgattggttcctcgacagcgctgcatcttgtgaggagtggttatgctcccgcaaatatcacggtcttggacacatttgagattccatcggctcaatcagccggccatgatctcaacaagatcatgggaatagatctgcgcaacaaggtggacctgcaaatgagtctagaggctagacagatgtggaaggaggatgagttattccagcccttctttcacaataccggcagaatggactgcgaacacacgcctgagggtatcgaggacctgaaaaagctgtaccagaaactgcacgatgccggtgcgggtctggagaagactcatgcctggttggacaacgaggatgagatcttatccaagatgccgttgcttcaacgtgaccaaatacaaggatggaaagcaatatggagtcaagatggcggctggttagctgcggcaaaggccatcaatgcgatcggacagttcttgaaagaacgtggtgtaaagttcggattcggcggcgctggatccttcaagcaaccccttttcgacgatgaaggcacaacttgcattggcgttgagacggcagatggtaccaaatattacgctgacaaggtggtcttagcagctggcgcatggagcccaaccctggtggacctggaagatcaatgttgctcgaaggcttgggtgtatgctcatattcagttgacgcctgaagaggccgctgagtataagggtgtcccagttgtgtataatggcgaatttggcttcttctttgagcctgatgagtttggtgtaataaaggtgtgcgacgagttcccaggattctcgcgcttcaaggaacatcaaccctatggcgccccatctccgaaacggatatcagtaccacgatcgcacgccaagcatcccacagacacttatccagacgcatccgaagtcagcatcaaaaaagcaatcgcgacgtttctccctcgatttcaggacaaggagctcttcaatcgcgccttgtgctggtgtacagacactgcggacgctgctctcttgatgtgtgaacaccccaaatggaagaatttcattctagcgaccggcgacagcggacactcattcaaaatcttgcctaacgtcggaaaatacgtagtcgagttgatagagggccgcctgccggaggaaatggcttatcaatggaggtggcggccaggaggcgatgcactcaagtctagacgtgcggcaccgccaaaagatcttgcagacatgccaggatggaaacatgatccgaaattgtaa

SEQ ID NO: 173 - protein, 437 aa, Coniochaeta sp.
MTSNRADTRVIVVGGGGTIGSSTALHLVRSGYAPANITVLDTFEIPSAQSAGHDLNKIMGIDLRNKVDLQMSLEARQMWKEDELFQPFFHNTGRMDCEHTPEGIEDLKKLYQRLHDAGAGLEKTHAWLDNEDEILSKMPLLQRDQIQGWKAIWSQDGGWLAAAKAINAIGQFLKERGVKFGFGGAGSFKQPLFDDEGTTCIGVETADGTKYYADKVVLAAGAWSPTLVDLEDQCCSKAWVYAHIQLTPEEAAEYKGVPVVYNGEFGFFFEPDEFGVIKVCDEFPGFSRFKEHQPYGAPSPKRISVPRSHAKHPTDTYPDASEVSIKKAIATFLPRFQDKELFNRALCWCTDTADAALLMCEHPKWKNFILATGDSGHSFKILPNVGKYVVELIEGRLPEEMAYQWRWRPGGDALKSRRAAPPKDLADMPGWKHDPKL

SEQ ID NO: 174 - DNA, 1314 bp, Coniochaeta sp.
atgacgtcgaatcgtgcagatacaagggtgattgtcgtcggtggcggaggaacgattggttcctcgacagcgctgcatcttgtgaggagtggttatgctcccgcaaatatcacggtcttggacacatttgagattccatcggctcaatcagccggccatgatctcaacaagatcatgggaatagatctgcgcaacaaggtggacctgcaaatgagtctagaggctagacagatgtggaaggaggatgagttattccagcccttctttcacaataccggcagaatggactgcgaacacacgcctgagggtatcgaggacctgaaaaagctgtaccagcgtctgcacgatgccggtgcgggtctggagaagactcatgcctggttggacaacgaggatgagatcttatccaagatgccgttgcttcaacgtgaccaaatacaaggatggaaagcaatatggagtcaagatggcggctggttagctgcggcaaaggccatcaatgcgatcggacagttcttgaaagaacgtggtgtaaagttcggattcggcggcgctggatccttcaagcaaccccttttcgacgatgaaggcacaacttgcattggcgttgagacggcagatggtaccaaatattacgctgacaaggtggtcttagcagctggcgcatggagcccaaccctggtggacctggaagatcaatgttgctcgaaggcttgggtgtatgctcatattcagttgacgcctgaagaggccgctgagtataagggtgtcccagttgtgtataatggcgaatttggcttcttctttgagcctgatgagtttggtgtaataaaggtgtgcgacgagttcccaggattctcgcgcttcaaggaacatcaaccctatggcgccccatctccgaaacggatatcagtaccacgatcgcacgccaagcatcccacagacacttatccagacgcatccgaagtcagcatcaaaaaagcaatcgcgacgtttctccctcgatttcaggacaaggagctcttcaatcgcgccttgtgctggtgtacagacactgcggacgctgctctcttgatgtgtgaacaccccaaatggaagaatttcattctagcgaccggcgacagcggacactcattcaaaatcttgcctaacgtcggaaaatacgtagtcgagttgatagagggccgcctgccggaggaaatggcttatcaatggaggtggcggccaggaggcgatgcactcaagtctagacgtgcggcaccgccaaaagatcttgcagacatgccaggatggaaacatgatccgaaattgtaa

SEQ ID NO: 175 - protein, 437 aa, Coniochaeta sp.
MTSNRADTRVIVVGGGGTIGSSTALHLVRSGYAPANITVLDTFEIPSAQSAGHDLNKIMGIDLRNKVDLQMSLEARQMWKEDELFQPFFHNTGRMDCEHTPEGIEKLKKLYQRLHDAGAGLEKTHAWLDNEDEILSKMPLLQRDQIQGWKAIWSQDGGWLAAAKAINAIGQFLKERGVKFGFGGAGSFKQPLFDDEGTTCIGVETADGTKYYADKVVLAAGAWSPTLVDLEDQCCSKAWVYAHIQLTPEEAAEYKGVPVVYNGEFGFFFEPDEFGVIKVCDEFPGFSRFKEHQPYGAPSPKRISVPRSHAKHPTDTYPDASEVSIKKAIATFLPRFQDKELFNRALCWCTDTADAALLMCEHPKWKNFILATGDSGHSFKILPNVGKYVVELIEGRLPEEMAYQWRWRPGGDALKSRRAAPPKDLADMPGWKHDPKL

SEQ ID NO: 176 - DNA, 1314 bp, Coniochaeta sp.
atgacgtcgaatcgtgcagatacaagggtgattgtcgtcggtggcggaggaacgattggttcctcgacagcgctgcatcttgtgaggagtggttatgctcccgcaaatatcacggtcttggacacatttgagattccatcggctcaatcagccggccatgatctcaacaagatcatgggaatagatctgcgcaacaaggtggacctgcaaatgagtctagaggctagacagatgtggaaggaggatgagttattccagcccttctttcacaataccggcagaatggactgcgaacacacgcctgagggtatcgagaaactgaaaaagctgtaccagcgtctgcacgatgccggtgcgggtctggagaagactcatgcctggttggacaacgaggatgagatcttatccaagatgccgttgcttcaacgtgaccaaatacaaggatggaaagcaatatggagtcaagatggcggctggttagctgcggcaaaggccatcaatgcgatcggacagttcttgaaagaacgtggtgtaaagttcggattcggcggcgctggatccttcaagcaaccccttttcgacgatgaaggcacaacttgcattggcgttgagacggcagatggtaccaaatattacgctgacaaggtggtcttagcagctggcgcatggagcccaaccctggtggacctggaagatcaatgttgctcgaaggcttgggtgtatgctcatattcagttgacgcctgaagaggccgctgagtataagggtgtcccagttgtgtataatggcgaatttggcttcttctttgagcctgatgagtttggtgtaataaaggtgtgcgacgagttcccaggattctcgcgcttcaaggaacatcaaccctatggcgccccatctccgaaacggatatcagtaccacgatcgcacgccaagcatcccacagacacttatccagacgcatccgaagtcagcatcaaaaaagcaatcgcgacgtttctccctcgatttcaggacaaggagctcttcaatcgcgccttgtgctggtgtacagacactgcggacgctgctctcttgatgtgtgaacaccccaaatggaagaatttcattctagcgaccggcgacagcggacactcattcaaaatcttgcctaacgtcggaaaatacgtagtcgagttgatagagggccgcctgccggaggaaatggcttatcaatggaggtggcggccaggaggcgatgcactcaagtctagacgtgcggcaccgccaaaagatcttgcagacatgccaggatggaaacatgatccgaaattgtaa

SEQ ID NO: 177 - protein, 437 aa, Coniochaeta sp.
MTSNRADTRVIVVGGGGTIGSSTALHLVRSGYAPANITVLDTFEIPSAQSAGHDLNKIMGIDARNKVDLQMSLEARQMWKEDELFQPFFHNTGRMDCEHTPEGIEKLKKLYQKLHDAGAGLEKTHAWLDNEDEILSKMPLLQRDQIQGWKAIWSQDGGWLAAAKAINAIGQFLKERGVKFGFGGAGSFKQPLFDDEGTTCIGVETADGTKYYADKVVLAAGAWSPTLVDLEDQCCSKAWVYAHIQLTPEEAAEYKGVPVVYNGEFGFFFEPDEFGVIKVCDEFPGFSRFKEHQPYGAPSPKRISVPRSHAKHPTDTYPDASEVSIKKAIATFLPRFQDKELFNRALCWCTDTADAALLMCEHPKWKNFILATGDSGHSFKILPNVGKYVVELIEGRLPEEMAYQWRWRPGGDALKSRRAAPPKDLADMPGWKHDPKL

SEQ ID NO: 178 - DNA, 1314 bp, Coniochaeta sp.
atgacgtcgaatcgtgcagatacaagggtgattgtcgtcggtggcggaggaacgattggttcctcgacagcgctgcatcttgtgaggagtggttatgctcccgcaaatatcacggtcttggacacatttgagattccatcggctcaatcagccggccatgatctcaacaagatcatgggaatagatgcgcgcaacaaggtggacctgcaaatgagtctagaggctagacagatgtggaaggaggatgagttattccagcccttctttcacaataccggcagaatggactgcgaacacacgcctgagggtatcgagaaactgaaaaagctgtaccagaaactgcacgatgccggtgcgggtctggagaagactcatgcctggttggacaacgaggatgagatcttatccaagatgccgttgcttcaacgtgaccaaatacaaggatggaaagcaatatggagtcaagatggcggctggttagctgcggcaaaggccatcaatgcgatcggacagttcttgaaagaacgtggtgtaaagttcggattcggcggcgctggatccttcaagcaaccccttttcgacgatgaaggcacaacttgcattggcgttgagacggcagatggtaccaaatattacgctgacaaggtggtcttagcagctggcgcatggagcccaaccctggtggacctggaagatcaatgttgctcgaaggcttgggtgtatgctcatattcagttgacgcctgaagaggccgctgagtataagggtgtcccagttgtgtataatggcgaatttggcttcttctttgagcctgatgagtttggtgtaataaaggtgtgcgacgagttcccaggattctcgcgcttcaaggaacatcaaccctatggcgccccatctccgaaacggatatcagtaccacgatcgcacgccaagcatcccacagacacttatccagacgcatccgaagtcagcatcaaaaaagcaatcgcgacgtttctccctcgatttcaggacaaggagctcttcaatcgcgccttgtgctggtgtacagacactgcggacgctgctctcttgatgtgtgaacaccccaaatggaagaatttcattctagcgaccggcgacagcggacactcattcaaaatcttgcctaacgtcggaaaatacgtagtcgagttgatagagggccgcctgccggaggaaatggcttatcaatggaggtggcggccaggaggcgatgcactcaagtctagacgtgcggcaccgccaaaagatcttgcagacatgccaggatggaaacatgatccgaaattgtaa

SEQ ID NO: 179 - protein, 437 aa, Coniochaeta sp.
MTSNRADTRVIVVGGGGTIGSSTALHLVRSGYAPANITVLDTFEIPSAQSAGHDLNKIMGIDHRNKVDLQMSLEARQMWKEDELFQPFFHNTGRMDCEHTPEGIEKLKKLYQKLHDAGAGLEKTHAWLDNEDEILSKMPLLQRDQIQGWKAIWSQDGGWLAAAKAINAIGQFLKERGVKFGFGGAGSFKQPLFDDEGTTCIGVETADGTKYYADKVVLAAGAWSPTLVDLEDQCCSKAWVYAHIQLTPEEAAEYKGVPVVYNGEFGFFFEPDEFGVIKVCDEFPGFSRFKEHQPYGAPSPKRISVPRSHAKHPTDTYPDASEVSIKKAIATFLPRFQDKELFNRALCWCTDTADAALLMCEHPKWKNFILATGDSGHSFKILPNVGKYVVELIEGRLPEEMAYQWRWRPGGDALKSRRAAPPKDLADMPGWKHDPKL

SEQ ID NO: 180 - DNA, 1314 bp, Coniochaeta sp.
atgacgtcgaatcgtgcagatacaagggtgattgtcgtcggtggcggaggaacgattggttcctcgacagcgctgcatcttgtgaggagtggttatgctcccgcaaatatcacggtcttggacacatttgagattccatcggctcaatcagccggccatgatctcaacaagatcatgggaatagatcatcgcaacaaggtggacctgcaaatgagtctagaggctagacagatgtggaaggaggatgagttattccagcccttctttcacaataccggcagaatggactgcgaacacacgcctgagggtatcgagaaactgaaaaagctgtaccagaaactgcacgatgccggtgcgggtctggagaagactcatgcctggttggacaacgaggatgagatcttatccaagatgccgttgcttcaacgtgaccaaatacaaggatggaaagcaatatggagtcaagatggcggctggttagctgcggcaaaggccatcaatgcgatcggacagttcttgaaagaacgtggtgtaaagttcggattcggcggcgctggatccttcaagcaaccccttttcgacgatgaaggcacaacttgcattggcgttgagacggcagatggtaccaaatattacgctgacaaggtggtcttagcagctggcgcatggagcccaaccctggtggacctggaagatcaatgttgctcgaaggcttgggtgtatgctcatattcagttgacgcctgaagaggccgctgagtataagggtgtcccagttgtgtataatggcgaatttggcttcttctttgagcctgatgagtttggtgtaataaaggtgtgcgacgagttcccaggattctcgcgcttcaaggaacatcaaccctatggcgccccatctccgaaacggatatcagtaccacgatcgcacgccaagcatcccacagacacttatccagacgcatccgaagtcagcatcaaaaaagcaatcgcgacgtttctccctcgatttcaggacaaggagctcttcaatcgcgccttgtgctggtgtacagacactgcggacgctgctctcttgatgtgtgaacaccccaaatggaagaatttcattctagcgaccggcgacagcggacactcattcaaaatcttgcctaacgtcggaaaatacgtagtcgagttgatagagggccgcctgccggaggaaatggcttatcaatggaggtggcggccaggaggcgatgcactcaagtctagacgtgcggcaccgccaaaagatcttgcagacatgccaggatggaaacatgatccgaaattgtaa

SEQ ID NO: 181 - protein, 437 aa, Coniochaeta sp.
MTSNRADTRVIVVGGGGTIGSSTALHLVRSGYAPANITVLDTFEIPSAQSAGHDLNKIMGIDHRNKVDLQMSLEARQMWKEDELFQPFFHNTGRMDCEHTPKGIEKLKKLYQKLHDAGAGLEKTHAWLDNEDEILSKMPLLQRDQIQGWKAIWSQDGGWLAAAKAINAIGQFLKERGVKFGFGGAGSFKQPLFDDEGTTCIGVETADGTKYYADKVVLAAGAWSPTLVDLEDQCCSKAWVYAHIQLTPEEAAEYKGVPVVYNGEFGFFFEPDEFGVIKVCDEFPGFSRFKEHQPYGAPSPKRISVPRSHAKHPTDTYPDASEVSIKKAIATFLPRFQDKELFNRALCWCTDTADAALLMCEHPKWKNFILATGDSGHSFKILPNVGKYVVELIEGRLPEEMAYQWRWRPGGDALKSRRAAPPKDLADMPGWKHDPKL

SEQ ID NO: 182 - DNA, 1314 bp, Coniochaeta sp.
atgacgtcgaatcgtgcagatacaagggtgattgtcgtcggtggcggaggaacgattggttcctcgacagcgctgcatcttgtgaggagtggttatgctcccgcaaatatcacggtcttggacacatttgagattccatcggctcaatcagccggccatgatctcaacaagatcatgggaatagatcatcgcaacaaggtggacctgcaaatgagtctagaggctagacagatgtggaaggaggatgagttattccagcccttctttcacaataccggcagaatggactgcgaacacacgcctaagggtatcgagaaactgaaaaagctgtaccagaaactgcacgatgccggtgcgggtctggagaagactcatgcctggttggacaacgaggatgagatcttatccaagatgccgttgcttcaacgtgaccaaatacaaggatggaaagcaatatggagtcaagatggcggctggttagctgcggcaaaggccatcaatgcgatcggacagttcttgaaagaacgtggtgtaaagttcggattcggcggcgctggatccttcaagcaaccccttttcgacgatgaaggcacaacttgcattggcgttgagacggcagatggtaccaaatattacgctgacaaggtggtcttagcagctggcgcatggagcccaaccctggtggacctggaagatcaatgttgctcgaaggcttgggtgtatgctcatattcagttgacgcctgaagaggccgctgagtataagggtgtcccagttgtgtataatggcgaatttggcttcttctttgagcctgatgagtttggtgtaataaaggtgtgcgacgagttcccaggattctcgcgcttcaaggaacatcaaccctatggcgccccatctccgaaacggatatcagtaccacgatcgcacgccaagcatcccacagacacttatccagacgcatccgaagtcagcatcaaaaaagcaatcgcgacgtttctccctcgatttcaggacaaggagctcttcaatcgcgccttgtgctggtgtacagacactgcggacgctgctctcttgatgtgtgaacaccccaaatggaagaatttcattctagcgaccggcgacagcggacactcattcaaaatcttgcctaacgtcggaaaatacgtagtcgagttgatagagggccgcctgccggaggaaatggcttatcaatggaggtggcggccaggaggcgatgcactcaagtctagacgtgcggcaccgccaaaagatcttgcagacatgccaggatggaaacatgatccgaaattgtaa

SEQ ID NO: 183 - protein, 437 aa, Coniochaeta sp.
MTSNRADTRVIVVGGGGTIGSSTALHLVRSGYAPANITVLDTFEIPSAQSAGHDLNKIMGIDHRNKVDLQMSLEARQMWKEDELFQPFFHNTGRMDCEHTPEGIEKLKKLYQKLHDAGAGLEKTHAWLDNEDEILSKMPLLQRDQIQGWKAIWSQDGGWLAAAKAINAIGQFLKERGVKFGFGGAGSFKQPLFDDEGTTCIGVETADGTKYYADKVVLAAGAWSPTLVDLEDQCCSKAWVYAHIQLTPEEAAEYKGVPVVYNGEFGFFFEPDEFGVIKVCDEFPGFSRFKEHQPYGAPSPKRISVPRSHAKHPTDTYPDASEVSIKKAIATFLPRFQDKELFNRALCWCTDTADAALLMCEHPKWKNFILATGDSGHSFKILPNVGKYVVELIEGRLPEEMAYQWRWRPGGDALKSRRKAPPKDLADMPGWKHDPKL

SEQ ID NO: 184 - DNA, 1314 bp, Coniochaeta sp.
atgacgtcgaatcgtgcagatacaagggtgattgtcgtcggtggcggaggaacgattggttcctcgacagcgctgcatcttgtgaggagtggttatgctcccgcaaatatcacggtcttggacacatttgagattccatcggctcaatcagccggccatgatctcaacaagatcatgggaatagatcatcgcaacaaggtggacctgcaaatgagtctagaggctagacagatgtggaaggaggatgagttattccagcccttctttcacaataccggcagaatggactgcgaacacacgcctgagggtatcgagaaactgaaaaagctgtaccagaaactgcacgatgccggtgcgggtctggagaagactcatgcctggttggacaacgaggatgagatcttatccaagatgccgttgcttcaacgtgaccaaatacaaggatggaaagcaatatggagtcaagatggcggctggttagctgcggcaaaggccatcaatgcgatcggacagttcttgaaagaacgtggtgtaaagttcggattcggcggcgctggatccttcaagcaaccccttttcgacgatgaaggcacaacttgcattggcgttgagacggcagatggtaccaaatattacgctgacaaggtggtcttagcagctggcgcatggagcccaaccctggtggacctggaagatcaatgttgctcgaaggcttgggtgtatgctcatattcagttgacgcctgaagaggccgctgagtataagggtgtcccagttgtgtataatggcgaatttggcttcttctttgagcctgatgagtttggtgtaataaaggtgtgcgacgagttcccaggattctcgcgcttcaaggaacatcaaccctatggcgccccatctccgaaacggatatcagtaccacgatcgcacgccaagcatcccacagacacttatccagacgcatccgaagtcagcatcaaaaaagcaatcgcgacgtttctccctcgatttcaggacaaggagctcttcaatcgcgccttgtgctggtgtacagacactgcggacgctgctctcttgatgtgtgaacaccccaaatggaagaatttcattctagcgaccggcgacagcggacactcattcaaaatcttgcctaacgtcggaaaatacgtagtcgagttgatagagggccgcctgccggaggaaatggcttatcaatggaggtggcggccaggaggcgatgcactcaagtctagacgtaaggcaccgccaaaagatcttgcagacatgccaggatggaaacatgatccgaaattgtaa

SEQ ID NO: 185 - protein, 438 aa, Aspergillus nidulans
MTPRANTKIIVVGGGGTMGSSTALHLLRAGYTPSNITVLDTCPIPSAQSAGYDLNKIMGIDHRNKPDLQLSLEALDMWKNDPLFKPFFHNVGMIDVSSTEKGIEKLRKLYQKLLDAGIGLEKTNFMLESEDEILAKAPHFTQEQIKGWKGLFCGDGGWLAAAKAINAIGQFLKEQGVKFGFGGAGTFKKPLFADAHEKTCIGVETVDGTKYYADKVVLAAGAWSSTLVDLEEQCVSKAWVFAHIQLTPAEAAAYKNTPVIYDGDYGFFFEPNENGIIKVCDEFPGFTHFKMHQPYGSPAPKPISVPRSHAKHPTDTYPHASEVTIKKAINRFLPRFNDKELFNRAMCWCTDTADSNLLVCEHPRWKGFYLATGDSGHSFKLLPNIGKHVVELLEERLESVFKDAWRWRPGSGDALKSRRAAPAKDLADMPGWRNEAKM

SEQ ID NO: 186 - DNA, 1317 bp, Aspergillus nidulans
atgacgccccgagccaacaccaaaatcattgtcgtcggcggcggcggcacaatgggctcgtcgacagccctacacctcctgcgcgccggctacacgccgtccaacattacagtgctcgacacgtgccctatcccctccgcacagtctgcaggctacgacctgaacaaaatcatgggcatcgatcatcgcaacaagcctgatttacagctctctcttgaggcgctggacatgtggaaaaatgatcctctcttcaagccgtttttccacaatgttggaatgatcgacgtctcttcaacagagaaaggcatcgagaaacttcggaagctgtaccagaaacttctcgacgcaggcattgggctcgagaagacgaatttcatgctggaaagtgaagacgagatcctggctaaagcgccgcatttcacgcaggagcagattaaaggctggaaaggcctgttctgtggcgacggcggctggctcgctgcagccaaagccatcaatgccattgggcagttcctcaaggaacagggcgtcaagtttggattcggcggcgccggcacgttcaaaaagccactcttcgccgatgcccacgagaagacgtgcatcggcgtcgagactgtagacggcacaaagtactacgccgacaaggtcgttctagcagctggtgcctggagttcgacgttggtcgatctggaggagcagtgcgtttcaaaggcctgggtctttgcccacatccaactgacgcccgctgaagcagccgcgtataagaacactcctgttatatacgacggtgactatgggtttttctttgagccgaatgaaaacggcatcataaaagtctgtgacgaattccctggcttcacgcatttcaaaatgcaccagccgtacggctcgccggcgcccaaacccatctctgtgcctcgttcccatgcgaagcaccccacagatacatacccgcacgcgtcggaggtcacgatcaaaaaggctatcaaccggttcctgccgaggttcaatgacaaggaactgtttaacagggccatgtgctggtgcaccgataccgcggatagcaatctgcttgtttgtgagcatccacgctggaaggggttttatcttgcaacaggggacagtgggcattcgttcaagttgctgccgaatattggaaagcatgttgtcgagttattggaggagaggctggaaagtgtgtttaaggatgcttggaggtggaggcctggcagtggggatgcattaaaaagtagacgggctgcgcctgcgaaggacctggcggatatgccggggtggaggaatgaggcaaagatgtag

SEQ ID NO: 187 - protein, 437 aa, Phaeosphaeria nodorum
MAPSRANTSVIVVGGGGTIGSSTALHLVRSGYTPSNVTVLDAYPIPSSQSAGNDLNKIMGVDHRNPVDLQLALEARQMWNEDELFKKFFHNTGRLDCAHGEKDIAKLKSLYQKLVDAGLDATNEWLDSEDEILKRMPLLSRDQIKGWKAIFSKDGGWLAAAKAINAVGEYLRDQGVRFGFYGAGSFKAPLLAEGVCIGVETVDGTRYYADKVVLAAGAWSPTLVELHEQCVSKAWVYGHIQLTPEEAARYKNSPVVYNGDVGFFFEPNEHGVIKVCDEFPGFTRFKMHQPFGAKAPKRISVPRSHAKHPTDTIPDASDVSIRRAIATFMPQFKNKKMFNQAMCWCTDTADSALLICEHPEWKNFVLATGDSGHSFKLLPNIGKHVVELLEGTLADDLAHAWRWRPGSGDALKSRRSAPAKDLADMPGWNHDKPRANL

SEQ ID NO: 188 - DNA, 1314 bp, Phaeosphaeria nodorum
atggccccgtcgcgtgctaatacgtcggtcattgtggttggtggtggtggtacgattggctcatctacggctctgcatctggtccgctcaggctataccccgtcgaacgtgacggttctggatgcatacccgattccgagctctcagagcgctggcaacgacctgaataaaatcatgggtgtcgatcatcgtaatccggtggatctgcagctggctctggaagcgcgccaaatgtggaacgaagacgaactgttcaagaagtttttccataacaccggccgtctggattgcgcgcacggtgaaaaagatattgccaaactgaagagcctgtatcagaaactggtggatgcgggtctggacgccacgaacgaatggctggatagtgaagacgaaatcctgaaacgtatgccgctgctgtcccgcgatcaaattaaaggctggaaggcgatcttttcaaaagacggtggttggctggcagcagcaaaggcaattaatgcagttggtgaatatctgcgtgatcagggcgtccgcttcggtttttacggcgccggttctttcaaagcaccgctgctggctgaaggcgtctgcatcggtgtcgaaaccgtggatggcacgcgctattacgcagacaaagtggttctggctgcaggtgcatggtcgccgaccctggttgaactgcatgaacagtgtgtgagcaaagcgtgggtttacggccacattcaactgacgccggaagaagccgcacgttataagaacagcccggtcgtgtacaatggcgatgtgggctttttctttgaaccgaacgaacatggcgttatcaaagtctgcgatgaatttccgggttttacccgcttcaagatgcaccagccgtttggtgccaaagcaccgaagcgtattagtgtgccgcgctcccatgccaaacacccgaccgatacgatcccggatgcaagtgacgtttccattcgtcgcgctatcgcgacctttatgccgcagttcaagaacaaaaagatgttcaaccaagcgatgtgctggtgtaccgatacggccgacagcgcgctgctgatttgtgaacatccggaatggaaaaactttgttctggcgaccggcgattcaggtcattcgttcaaactgctgccgaatatcggcaagcacgttgtcgaactgctggagggtacgctggcagatgacctggcacacgcatggcgttggcgtccgggtagtggtgatgcactgaaaagccgtcgctctgctccggcgaaagacctggctgatatgccgggctggaaccatgacaaaccgcgtgctaatctgtaa

SEQ ID NO: 189 - protein, 443 aa, Cryptococcus neoformans
MPPSRASTKVIVIGGGGTLGSSTALHLLRAGYTPSNITVLDTYLIPSAQSAGNDLNKIMGIDIRNPVDKQLSLEARDMWRNDEVFKPYFHNTGRLDCAHTPESIAKLRKLYEKILKAGSGLEKTHHWLSTEDEILARAPLLDRKQIKGWKAIYSEDGGWLAAAKAINSIGQVLKEKGVTFGFGSAGSFKKPLFDEDGTKAIGIETVDGTQYFADKVVLAAGAWSPTLVDLEGQCCSKAWVYAHMQLTPEEAAEYKECPVVYNSELGFFFEPNEKGVIKVCDEFPGFTRFKQHQPYGASSTKHISFPRSHAKHPTDTIPDESDASIRRAISAFLPRFKEKELFNRALCWCTDTADANLLICEHPKWKNFILATGDSGHSFKILPNIGKHVVELIEGTLAEDLAESWRWRPGSGDPLISRRAAPARDLADLPGWNHDEPSDDDMD

SEQ ID NO: 190 - DNA, 1332 bp, Cryptococcus neoformans
atgccgccgtcccgtgcttcaacgaaagtgattgtcattggtggtggtggtacgctgggctcctcaaccgccctgcatctgctgcgcgcgggctataccccgagtaacattaccgtgctggatacgtacctgatcccgagtgcccagtccgcaggcaacgacctgaataaaattatgggtattgatatccgcaatccggtggataaacaactgagcctggaagcccgtgatatgtggcgcaacgacgaagttttcaaaccgtacttccataacaccggtcgtctggactgcgctcacacgccggaatcaattgcgaaactgcgtaaactgtacgaaaaaatcctgaaagcaggctcaggtctggaaaaaacccatcactggctgtcgacggaagatgaaatcctggcacgtgcaccgctgctggaccgtaaacagattaaaggttggaaagcaatctatagtgaagatggcggttggctggcggccgcaaaagctattaactccatcggccaagtcctgaaagaaaaaggtgtgaccttcggctttggtagcgcaggctcttttaaaaaaccgctgttcgatgaagacggcacgaaagccattggtatcgaaaccgttgatggtacgcagtattttgccgacaaagtggttctggctgcaggtgcatggagcccgaccctggttgatctggaaggccagtgctgttctaaagcttgggtctacgcgcacatgcaactgacgccggaagaagccgcagaatataaagaatgcccggtcgtgtacaacagcgaactgggctttttctttgaaccgaacgaaaaaggtgtgatcaaagtttgtgatgaattcccgggctttacccgtttcaaacagcatcaaccgtacggtgctagctctacgaaacacattagctttccgcgctctcatgcgaaacacccgaccgatacgatcccggatgaaagtgacgcctccattcgtcgcgctatctctgcgtttctgccgcgtttcaaagaaaaagaactgtttaaccgcgcgctgtgctggtgtaccgatacggctgacgcgaacctgctgatttgtgaacacccgaaatggaaaaattttatcctggccaccggcgattcaggtcattcgttcaaaattctgccgaatatcggcaaacacgttgtcgaactgattgaaggtaccctggccgaagatctggcagaaagctggcgttggcgtccgggcagtggtgacccgctgatctcccgtcgcgctgcgccggcgcgcgacctggcggacctgccgggctggaaccacgacgaaccgagcgacgatgacatggactga

SEQ ID NO: 191 - protein, 440 aa, Curvularia clavata
MAPSRANTSVIVVGGGGTIGSSTALHLVRSGYTPSNITVLDAYPIPSSQSAGNDLNKIMGIDHRNKVDLQLSLEARQMWREDDLFKEYFHNTGRLDCAHGEEGLAKLRQLYQKLLDANAGLEETTEWLDSEDEILKKMPLLSRDQIKGWKAVYSQDGGWLAAAKAINAIGEYLRAQGVKFGFGGAGSFKQPLLAEGVCIGVETVDGTRYYADKVVLAAGAWSPTLVELHEQCVSKAWVYGHIQLTPEEAAEYKNSPVVYNGDVGFFFEPNEHGVIKVCDEFPGFTRFKMHQPFGAKAPKRISVPRSHAKHPTDTIPDASEKSIRKAIATFLPKFTEKELFNRHLCWCTDTADSALLICEHPEWKNFVLATGDSGHSFKLLPNIGKHVVELLEGTLADDLAHAWRWRPGSGDALKSRRSAPAKDLADMPGWKHDDVVKSKL

SEQ ID NO: 192 - DNA, 1323 bp, Curvularia clavata
atggccccgtcgcgtgctaatacgtcggtcattgtggttggtggtggtggtacgattggctcatctacggctctgcatctggtccgctcaggctataccccgtcgaacattacggttctggatgcatacccgattccgagctctcagagcgctggcaacgacctgaataaaatcatgggtatcgatcatcgtaataaggtggatctgcagctgtctctggaagcgcgccaaatgtggcgcgaagacgatctgttcaaggagtatttccataacaccggccgtctggattgcgcgcacggtgaagaaggtcttgccaaactgcgtcaactgtatcagaaactgctggatgcgaatgcgggtctggaagagacgaccgaatggctggatagtgaagacgaaatcctgaaaaaaatgccgctgctgtcccgcgatcaaattaaaggctggaaggcggtgtattcacaggacggtggttggctggcagcagcaaaggcaattaatgcaattggtgaatatctgcgtgctcagggcgtcaaattcggttttggcggcgccggttctttcaaacaaccgctgctggctgaaggcgtctgcatcggtgtcgaaaccgtggatggcacgcgctattacgcagacaaagtggttctggctgcaggtgcatggtcgccgaccctggttgaactgcatgaacagtgtgtgagcaaagcgtgggtttacggccacattcaactgacgccggaagaagccgcagaatataagaacagcccggtcgtgtacaatggcgatgtgggctttttctttgaaccgaacgaacatggcgttatcaaagtctgcgatgaatttccgggttttacccgcttcaagatgcaccagccgtttggtgccaaagcaccgaagcgtattagtgtgccgcgctcccatgccaaacacccgaccgatacgatcccggatgcaagtgaaaaatccattcgtaaagctatcgcgacctttctgccgaagttcacggagaaagagctgttcaaccgtcatctgtgctggtgtaccgatacggccgacagcgcgctgctgatttgtgaacatccggaatggaaaaactttgttctggcgaccggcgattcaggtcattcgttcaaactgctgccgaatatcggcaagcacgttgtcgaactgctggagggtacgctggcagatgacctggcacacgcatggcgttggcgtccgggtagtggtgatgcactgaaaagccgtcgctctgctccggcgaaagacctggctgatatgccgggctggaaacatgacgatgtggtgaaaagcaaactgtaa

SEQ ID NO: 193 - DNA, 28 bp, Artificial
  primer
caccttgttgcgatgatctattcccatg

SEQ ID NO: 194 - DNA, 28 bp, Artificial
  primer
cgcaacaaggtgaacctgcaaatgagtc

SEQ ID NO: 195 - DNA, 28 bp, Artificial
  primer
agagtccgcagtgtctgtacaccagcac

SEQ ID NO: 196 - DNA, 30 bp, Artificial
  primer
acactgcggactctactctcttgatgtgtg

SEQ ID NO: 197 - DNA, 10 bp, Artificial
  primer
aaaaaaaaaa

SEQ ID NO: 198 - DNA, 10 bp, Artificial
  primer
cccccccccc

SEQ ID NO: 199 - protein, 434 aa, Coniochaeta sp. NISL 9330
MTSNRADTRVIVVGGGGTIGSSTALHLVRSGYAPANITVLDTFPIPSAQSAGHDLNKIMGIDHRNKVNLQMSLEARQMWKEDELFQPFFHNTGRMDCEHTPKGIEKLKKLYQKLHDAGAGLEKTHAWLDNEDAILSKMPLLQRDQIQGWKAIWSQDGGWLAAAKAINAIGQFLKERGVKFGFGGAGSFKQPLFDDEGTTCIGVETADGTKYYADKVVLAAGAWSPTLVDLEDQCCSKAWVYAHIQLTPEEAAKYKGCPVVYHGEFGFFFEPDEFGVIKVCDEFPGFSRFKEHQPYGAPSPKRISVPRSHAKHPTDTYPDASEVSIKKAIATFLPRFKDKPLFNRALCWCTDTADSALLMCEHPKWKNFILATGDSGHSFKILPNVGKYVVELIEGRLPEEMAYQWRWRPGGDALKSRRAAPPKDLADMPGWKHD

SEQ ID NO: 200 - DNA, 1305 bp, Coniochaeta sp. NISL 9330
atgacctcaaaccgtgctgatacccgtgttattgttgttggtggtggtggtacgattggctcctcgaccgctctgcatctggtgcgtagtggctatgctccggcgaacattaccgtcctggatacgtttccgatcccgagcgcccagtctgcaggccatgatctgaataaaattatgggtatcgaccaccgtaacaaagttaatctgcagatgagcctggaagcgcgccaaatgtggaaagaagatgaactgttccagccgtttttccataacaccggccgtatggactgcgaacacacgccgaaaggtatcgaaaaactgaaaaaactgtaccaaaaactgcatgatgccggcgcaggtctggaaaaaacccacgcctggctggataacgaagacgcaattctgagcaaaatgccgctgctgcagcgtgatcagattcaaggttggaaagccatctggtctcaagacggcggttggctggcagcagcaaaagctattaatgcgatcggccagtttctgaaagaacgcggcgtgaaattcggttttggcggtgcaggttcttttaaacaaccgctgttcgatgacgaaggcaccacgtgtatcggtgttgaaaccgctgatggcacgaaatattacgcggacaaagtggttctggctgcaggtgcatggagtccgaccctggtcgatctggaagaccagtgctgttccaaagcgtgggtgtatgcgcatattcaactgacgccggaagaagccgcaaaatataaaggctgcccggtcgtgtaccacggcgaatttggctttttctttgaaccggatgaatttggcgtgatcaaagtttgtgacgaatttccgggtttttcacgtttcaaagaacatcagccgtatggtgcgccgtcgccgaaacgtattagcgttccgcgctctcatgccaaacacccgaccgatacgtacccggacgcaagtgaagtctccattaagaaagcgatcgcgacctttctgccgcgtttcaaagataaaccgctgtttaatcgcgcactgtgctggtgtaccgatacggccgacagcgcactgctgatgtgcgaacatccgaaatggaaaaactttattctggcgaccggcgattcaggtcactcgttcaaaatcctgccgaatgtgggcaaatatgttgtcgaactgattgaaggtcgcctgccggaagaaatggcttaccagtggcgttggcgtccgggcggtgatgccctgaaaagtcgccgtgctgctccgccgaaagacctggctgatatgccgggctggaaacatgactaa

SEQ ID NO: 201 - DNA, 30 bp, Artificial
  primer
gctgtcggccgtatcggtacaccagcacag

SEQ ID NO: 202 - DNA, 30 bp, Artificial
  primer
atacggccgacagcacactgctgatgtgcg

SEQ ID NO: 203 - protein, 434 aa, Coniochaeta sp.
MTSNRADTRVIVVGGGGTIGSSTALHLVRSGYAPANITVLDTFPIPSAQSAGHDLNKIMGIDHRNKVNLQMSLEARQMWKEDELFQPFFHNTGRMDCEHTPKGIEKLKKLYQKLHDAGAGLEKTHAWLDNEDAILSKMPLLQRDQIQGWKAIWSQDGGWLAAAKAINAIGQFLKERGVKFGFGGAGSFKQPLFDDEGTTCIGVETADGTKYYADKVVLAAGAWSPTLVDLEDQCCSKAWVYAHIQLTPEEAAKYKGCPVVYHGEFGFFFEPDEFGVIKVCDEFPGFSRFKEHQPYGAPSPKRISVPRSHAKHPTDTYPDASEVSIKKAIATFLPRFKDKPLFNRALCWCTDTADSTLLMCEHPKWKNFILATGDSGHSFKILPNVGKYVVELIEGRLPEEMAYQWRWRPGGDALKSRRAAPPKDLADMPGWKHD

SEQ ID NO: 204 - DNA, 1305 bp, Coniochaeta sp.
atgacctcaaaccgtgctgatacccgtgttattgttgttggtggtggtggtacgattggctcctcgaccgctctgcatctggtgcgtagtggctatgctccggcgaacattaccgtcctggatacgtttccgatcccgagcgcccagtctgcaggccatgatctgaataaaattatgggtatcgaccaccgtaacaaagttaatctgcagatgagcctggaagcgcgccaaatgtggaaagaagatgaactgttccagccgtttttccataacaccggccgtatggactgcgaacacacgccgaaaggtatcgaaaaactgaaaaaactgtaccaaaaactgcatgatgccggcgcaggtctggaaaaaacccacgcctggctggataacgaagacgcaattctgagcaaaatgccgctgctgcagcgtgatcagattcaaggttggaaagccatctggtctcaagacggcggttggctggcagcagcaaaagctattaatgcgatcggccagtttctgaaagaacgcggcgtgaaattcggttttggcggtgcaggttcttttaaacaaccgctgttcgatgacgaaggcaccacgtgtatcggtgttgaaaccgctgatggcacgaaatattacgcggacaaagtggttctggctgcaggtgcatggagtccgaccctggtcgatctggaagaccagtgctgttccaaagcgtgggtgtatgcgcatattcaactgacgccggaagaagccgcaaaatataaaggctgcccggtcgtgtaccacggcgaatttggctttttctttgaaccggatgaatttggcgtgatcaaagtttgtgacgaatttccgggtttttcacgtttcaaagaacatcagccgtatggtgcgccgtcgccgaaacgtattagcgttccgcgctctcatgccaaacacccgaccgatacgtacccggacgcaagtgaagtctccattaagaaagcgatcgcgacctttctgccgcgtttcaaagataaaccgctgtttaatcgcgcactgtgctggtgtaccgatacggccgacagcacactgctgatgtgcgaacatccgaaatggaaaaactttattctggcgaccggcgattcaggtcactcgttcaaaatcctgccgaatgtgggcaaatatgttgtcgaactgattgaaggtcgcctgccggaagaaatggcttaccagtggcgttggcgtccgggcggtgatgccctgaaaagtcgccgtgctgctccgccgaaagacctggctgatatgccgggctggaaacatgactaa